European Patent Application EP 4 361 265 A1, published May 1, 2024. Title: Optimization of editing efficacy of CRISPR nucleases with collateral activity. Applicant: BRAIN Biotech AG. The sequence listing filed with the application follows.

SEQUENCE LISTING (40 sequences)

SEQ ID NO: 1 - protein, 1231 aa, synthetic construct
  REGION 1..1231: note = BEC85 AA Sequence
MKSFENSCQISKTLRFGATLKEDKKKCKSHLELQEFVDISYKTLKSSATIAESLNEIELVKKCERCYSEIIKFHEAWGQIYCRTNQIAVYKDWYRQLARKARFDVGDQNSQLITLSSLSSKHNVYQGLKRSQHITNYWKDNIARQKSFLKDFSQQLKQYKRALENSDKAHTKPNLINFNKTFSILANLVNEIVIPLSNGAISFPNISKLEDGEESRHLIEFALNDYSDLVGSIGELKDAIATNGGYTPFAKVTLNHYTAEQKPHVFKNDIDAKIRELKLIELVEKLKNKTSKQIEEYFSKFDKFKIYDDRNISVIIRTQCFKYKPIPFLVKHELAKYIAEDEDAVLKVLDAIGATRSPAHDYAHNEDVFDLNHYPIKVAFDYAWEQLANSLYTTVTFPKEQCEKYLKDVFDCEVSKEPVFKFYADLLYIRKNLAVLEHKNNLPSNQEEFICKINNTFENIVLPYKISQFETYKKDILAWINDGRGHEKYTDAKQQLGFIRGGLKGRIKAQKMFRKDKYGKIKSYYENPYTKLTNEFKQISSTYGKTFAELRDKFKEKNNITKITHFGIIIEDKNRDRYLLANGLQHEQINHVSTILNKLDKSSEFITYQVKSLTSKTLIKLIKNHTTKKGAISPYADFHTSKTGFNKNEIEKNWDNYKREQVLVEYVKDCLTDSTMAKNQNWAEFGWNFEKCNSYEDIEHEIDQKSYILQKHTISKQSIASLVEGGCLLLPIINQDITSKERKDKNQFSKDWKQIFEGSKEFRLHPEFAVSYRTPIEGYPVQKRYGRLQFVCAFNCEIIPQNGEFINLKKQIENFNDEDAQKEAVEEFNKKVNHALSDKEYVVIGIDRGLKQLATLCVLDKRGKILGDFEIYKKEFVRAEKRSESHWEHTQAETRHILDLSNLRVETTIEGKKVLVDQSLTLVKKNRDTPDEEATEENKQKIKLKQLSYIRKLQHKMQTNEQDVLDLINNEPSDEEFKKRIEGLISSFGEGQKYADLPINTMREMISDLQGVIARGNNQTEKNKIIELDAADNLKQGIVANMIGIVNYIFAKYSYKAYISLEDLSRAYGGAKSGYDGRYLPSTSQDEDVDFKEQQNQMLAGLGTYQFFEMQLLKKLQKIQSDNTVLRFVPAFRSADNYRNILRLEETKYKSKPFGVVHFIDPKFTSKKCPVCSKTNVYRDKDDILVCKECGFRSDSQLKERENNIHYIHNGDDNGAYHIALKSVENLIQMK

SEQ ID NO: 2 - protein, 1231 aa, synthetic construct
  REGION 1..1231: note = BEC67 AA Sequence
MKSFENSCQISKTLRFGATLKEDKKKCKSHLELQEFVDISYKTLKSSATIAESLNEIELVKKCERCYSEIIKFHEAWGQIYCRTNQIAVYKDWYRQLARKARFDVGDQNSQLITLSSLSSKHNVYQGLKRSQHITNYWKDNIARQKSFLKDFSQQLKQYKRALENSDKAHTKPNLINFNKTFSILANLVNEIVIPLSNGAISFPNISKLEDGEESRHLIEFALNDYSDLVGSIGELKDAIATNGGYTPFAKVTLNHYTAEQKPHVFKNDIDAKIRELKLIELVEKLKNKTSKQIEEYFSKFDKFKIYDDRNISVIIRTQCFKYKPIPFLVKHELAKYIAEDEDAVLKVLDAIGATRSPAHDYAHNEDVFDLNHYPIKVAFDYAWEQLANSLYTTVTFPKEQCEKYLKDVFDCEVSKEPVFKFYADLLYIRKNLAVLEHKNNLPSNQEEFICKINNTFENIVLPYKISQFETYKKDILAWINDGRGHEKYTDSKRELGFIRGGLKGRIKAQKMFRKDKYGKIKSYYENPYTKLTEEFKNLAITYGKTFAELRDKFKEKNNITKITHFGIIIEDKNRDRYLLANGLQHEQINHVSTILNKLDKSSEFITYQVKSLTSKTLIKLIKNHTTKKGAISPYADFHTSKTGFNKNEIEKNWDNYKREQVLVEYVKDCLTDSTMAKNQNWAEFGWDLESCNSYEDIEHEIDQKSYILQKHTISKQSIASLVEGGCLLLPIINQDITSKERKDKNQFSKDWKQIFEGSKEFRLHPEFAVSYRTPIEGYPVQKRYGRLQFVCAFNCEIIPQNGEFINLKKQIENFNDEDAQKEAVEEFNKKVNHALSDKEYVVIGIDRGLKQLATLCVLDKRGKILGDFEIYKKEFVRAEKRSESHWEHTQAETRHILDLSNLRVETTIEGKKVLVDQSLTLVKKNRDTPDEEATEENKQKIKLKQLSYIRKLQHKMQTNEQDVLDLINNEPSDEEFKKRIEGLISSFGEGQKYADLPINTMREMISDLQGVIARGNNQTEKNKIIELDAADNLKQGIVANMIGIVNYIFAKYSYKAYISLEDLSRAYGGAKSGYDGRYLPSTSQDEDVDFKEQQNQMLAGLGTYQFFEMQLLKKLQKIQSDNTVLRFVPAFRSADNYRNILRLEETKYKSKPFGVVHFIDPKFTSKKCPVCSKTNVYRDKDDILVCKECGFRSDSQLKERENNIHYIHNGDDNGAYHIALKSVENLIQMK

SEQ ID NO: 3 - protein, 1231 aa, synthetic construct
  REGION 1..1231: note = BEC10 AA Sequence
MKSFENSCQISKTLRFGATLKEDKKKCKSHLELQEFVDISYKTLKSSATIAESLNEIELVKKCERCYSEIIKFHEAWGQIYCRTNQIAVYKDWYRQLARKARFDVGDQNSQLITLSSLSSKHNVYQGLKRSQHITNYWKDNIARQKSFLKDFSQQLKQYKRALENSDKAHTKPNLINFNKTFSILANLVNEIVIPLSNGAISFPNISKLEDGEESRHLIEFALNDYSDLVGSIGELKDAIATNGGYTPFAKVTLNHYTAEQKPHVFKNDIDAKIRELKLIELVEKLKNKTSKQIEEYFSKFDKFKIYDDRNISVIIRTQCFKYKPIPFLVKHELAKYIAEDEDAVLKVLDAIGATRSPAHDYAHNEDVFDLNHYPIKVAFDYAWEQLANGVYTTVTFPKEQCEKYLKDVFDCEVSKEPVFKFYADLLYIRKNLAVLEHKNNLPSNQEEFICKINNTFENIVLPYKIKEFETYKKDILAWINDGRGHEKYTDAKQQLGFIRGGLKGRIKAQKMFRKDKYGKIKSYYENPYTKLTNEFKQISSTYGKTFAELRDKFKEKNNITKITHFGIIIEDNNKDRYLLANGLQHEQINHVEAILGKLNTSSEFITYQVKSLTSKTLIKLIKNHTTKKGAISPYADFHTSKIHVDWTKIKKEWDNYKREQVLLQYVKDCLTDSTMAKNQNWAEFGWNFEKCNSYEDIEHEIDQKSYILQKHTISKQSIASLVEGGCLLLPIINQDITSQGRKDKNQFSKDWKQIFEGSKEFRLHPEFAVSYRTPIKDYPKDKRYGRLQFVCAFNCEIIPQNGEFINLKKQIENFNDEDAQKEAVEEFNKKVNHALLGKEYVVIGIDRGLKQLATLCVLDKRGKILGDFEIYKKEFVRAEKRSKNYWKHTLAETRHILDLSNLRVETTIEDNKVLVDQSLTLVKKNRDTPDEEATEENKQKIKLKQLSYIRKLQHKMQTNEQDVLDLINNEPSDEEFKKRIEGLISSFGEGQKYADLPINTMREMISDLQGVIARGNNQTEKNKIIELDAADNLKQGIVANMIGIVNYIFAKYSYKAYISLEDLSRAYGGAKSGYDGRYLPSTSQDEDVDFKEQQNQMLAGLGTYQFFEMQLLKKLQKIQSDNTVLRFVPAFRSADNYRNIIKLEETKYKSKPFGVVHFIDPKFTSKKCPVCSKTNVYRDKDDILVCKECGFRSDSQLKERENNIHYIHNGDDNGAYHIALKSVENLIQMK

SEQ ID NO: 4 - DNA, 3696 bp, synthetic construct
  misc_feature 1..3696: note = BEC85 NT Sequence (Yeast codon optimized)
  source 1..3696: mol_type = other DNA
atgaagtccttcgaaaactcctgccaaatttctaagactttgagattcggtgccactttgaaagaggataagaaaaagtgcaagtcccacttggaattgcaagaattcgttgacatttcctacaagaccttgaagtcatctgctaccattgctgaatccttgaacgaaatcgaattggtcaaaaagtgcgaaaggtgctactccgaaattatcaagttccatgaagcttggggtcaaatctactgtagaactaaccaaattgccgtctacaaggactggtatagacaattggctagaaaggccagattcgatgttggtgatcaaaactctcaactgatcaccttgtcatccttatcttctaagcacaacgtttaccagggtttgaagagatctcaacatattaccaactactggaaggacaacattgccagacaaaagtctttcctgaaggatttctctcaacaattgaagcagtacaagagagctttggaaaattctgataaggctcataccaagccaaacctgattaacttcaacaagaccttctccattttggccaacttggttaacgaaattgtcatcccattgtccaacggtgctatttcttttccaaacatctccaagttggaagatggtgaagaatccagacatttgattgaattcgctctgaacgattactccgatttggttggttctattggtgaattgaaggatgctattgctaccaatggtggttatactccatttgctaaggttaccttgaaccattacactgctgaacaaaagccacacgttttcaagaacgatattgatgccaagatccgtgagttgaagttgattgagttggtcgaaaagttgaagaacaagacgtccaagcaaatcgaagagtacttttccaagttcgacaagttcaagatctacgatgatagaaacatctccgttatcattagaacccaatgctttaagtacaagcccattccatttttggtcaagcacgaattggctaagtatatcgctgaagatgaagatgccgttttgaaggttttggatgcaattggtgctactagatctccagctcatgattacgctcataatgaagatgtttttgacttgaatcactacccaatcaaggttgcttttgattacgcatgggaacaattggctaactccttgtacactactgttactttcccaaaagaacagtgcgagaagtacttgaaggatgtttttgattgcgaagtctccaaagaaccagtttttaagttctacgccgacctgttgtacatcagaaagaatttggctgttttggagcacaagaacaacctgccatctaatcaagaggaattcatctgcaagattaacaacaccttcgagaacatcgttctgccatacaagatttctcaattcgaaacctacaagaaggatatcttggcctggattaacgatggtagaggtcacgaaaagtacaccgatgctaaacaacagttgggttttattagaggtggtctgaaaggtagaatcaaggctcaaaagatgttcagaaaagacaagtacggtaagatcaagtcctactacgaaaacccatacactaagttgaccaacgaattcaagcaaatctcttctacctacggtaaaaccttcgctgaattgagagacaagttcaaagaaaagaacaacatcaccaagatcacccatttcggtattatcatcgaagataagaacagggacagatacttgttggccaacggtttgcaacacgaacaaatcaaccatgtctccaccatcttgaacaagttggataagtcatccgaattcatcacctaccaagttaagtctttgacctctaagaccctgatcaagctgattaagaatcataccaccaagaagggtgcaatttctccatatgctgatttccatacttctaagaccggctttaacaaaaacgagatcgaaaagaactgggacaactacaagagagaacaagtcttggttgaatacgttaaggattgcttgaccgattctaccatggctaagaatcaaaattgggctgaatttggttggaacttcgagaagtgtaactcctacgaagatatcgaacacgaaatcgatcagaagtcttacatcttgcaaaagcataccatttccaagcaatctattgcttctttggttgaaggtggttgtttgttgttgccaattatcaaccaggacatcacctctaaagaacgtaaggacaagaatcagttctccaaggattggaagcaaatcttcgaaggttccaaagaattcagattgcatccagaattcgccgtttcttacagaactccaattgaaggttacccagtccaaaaaagatacggtagattgcaattcgtttgcgcttttaactgcgaaatcatcccacaaaatggtgagttcatcaacttgaagaagcagatcgagaacttcaacgacgaagatgctcaaaaagaagccgtcgaagagttcaacaaaaaggttaaccatgccttgtccgacaaagaatacgttgttattggtatcgacagaggcttgaagcaattagctactttgtgtgttttggacaagaggggtaagattttgggtgactttgaaatctacaaaaaagagttcgtcagagccgaaaagagatctgaatctcattgggaacatactcaagctgaaaccagacatatcttggacttgtctaacttgagagttgaaactaccattgagggcaaaaaggtgttggttgatcaatctttgacactggtcaagaagaacagagatactccagatgaagaagctaccgaagaaaacaagcagaagattaagttgaagcagctgtcctacattagaaagttgcaacacaagatgcagaccaatgaacaagatgtcttggacctgatcaacaacgaaccatctgatgaagaattcaaaaagaggatcgagggcttgatttcttcattcggtgaaggtcaaaagtacgctgatttgcctattaacaccatgagggaaatgatctctgacttgcaaggtgttattgccagaggaaacaatcagactgagaaaaacaagatcatcgaattggatgctgccgacaatttgaaacaaggtatcgttgctaacatgatcggtatcgttaactacattttcgccaagtactcctacaaggcctacatttctttagaagatttgtccagagcttacggtggtgcaaaatctggttatgatggtagatatttgccatccacctctcaagatgaggatgttgactttaaagaacagcagaatcaaatgttggctggcttgggtacttaccaattttttgaaatgcagctgctgaaaaagctgcagaagatccaatctgataacaccgttttgagatttgttccagcttttagatccgccgataactacagaaatatcttgagattggaagagactaagtacaagtctaagccattcggtgttgttcatttcatcgatccaaagttcacatctaagaagtgtccagtttgctctaagactaacgtttacagagataaggatgacatcctggtctgtaaagaatgtggttttaggtccgactcacagttgaaagaaagggaaaacaacatccactacatccacaatggtgatgataatggtgcttaccatattgccttgaagtccgtcgaaaacttgattcagatgaagtaa

SEQ ID NO: 5 - DNA, 3696 bp, synthetic construct
  misc_feature 1..3696: note = BEC67 NT Sequence (Yeast codon optimized)
  source 1..3696: mol_type = other DNA
atgaagtccttcgaaaactcctgccaaatttctaagactttgagattcggtgccactttgaaagaggataagaaaaagtgcaagtcccacttggaattgcaagaattcgttgacatttcctacaagaccttgaagtcatctgctaccattgctgaatccttgaacgaaatcgaattggtcaaaaagtgcgaaaggtgctactccgaaattatcaagttccatgaagcttggggtcaaatctactgtagaactaaccaaattgccgtctacaaggactggtatagacaattggctagaaaggccagattcgatgttggtgatcaaaactctcaactgatcaccttgtcatccttatcttctaagcacaacgtttaccagggtttgaagagatctcaacatattaccaactactggaaggacaacattgccagacaaaagtctttcctgaaggatttctctcaacaattgaagcagtacaagagagctttggaaaattctgataaggctcataccaagccaaacctgattaacttcaacaagaccttctccattttggccaacttggttaacgaaattgtcatcccattgtccaacggtgctatttcttttccaaacatctccaagttggaagatggtgaagaatccagacatttgattgaattcgctctgaacgattactccgatttggttggttctattggtgaattgaaggatgctattgctaccaatggtggttatactccatttgctaaggttaccttgaaccattacactgctgaacaaaagccacacgttttcaagaacgatattgatgccaagatccgtgagttgaagttgattgagttggtcgaaaagttgaagaacaagacgtccaagcaaatcgaagagtacttttccaagttcgacaagttcaagatctacgatgatagaaacatctccgttatcattagaacccaatgctttaagtacaagcccattccatttttggtcaagcacgaattggctaagtatatcgctgaagatgaagatgccgttttgaaggttttggatgcaattggtgctactagatctccagctcatgattacgctcataatgaagatgtttttgacttgaatcactacccaatcaaggttgcttttgattacgcatgggaacaattggctaactccttgtacactactgttactttcccaaaagaacagtgcgagaagtacttgaaggatgtttttgattgcgaagtctccaaagaaccagtttttaagttctacgccgacctgttgtacatcagaaagaatttggctgttttggagcacaagaacaacctgccatctaatcaagaggaattcatctgcaagattaacaacaccttcgagaacatcgttctgccatacaagatttctcaattcgaaacctacaagaaggatatcttggcctggattaacgatggtagaggtcacgaaaagtacaccgattctaaaagagaattgggttttattagaggtggtctgaaaggtagaatcaaggctcaaaagatgttcagaaaagacaagtacggtaagatcaagtcctactacgaaaacccatacactaagttgaccgaagagttcaagaacttggccatcacctacggtaaaaccttcgctgaattgagagacaagttcaaagaaaagaacaacatcaccaagatcacccatttcggtattatcatcgaagataagaacagggacagatacttgttggccaacggtttgcaacacgaacaaatcaaccatgtctccaccatcttgaacaagttggataagtcatccgaattcatcacctaccaagttaagtctttgacctctaagaccctgatcaagctgattaagaatcataccaccaagaagggtgcaatttctccatatgctgatttccatacttctaagaccggctttaacaaaaacgagatcgaaaagaactgggacaactacaagagagaacaagtcttggttgaatacgttaaggattgcttgaccgattctaccatggctaagaatcaaaattgggctgaatttggttgggatttggagtcttgtaactcctacgaagatatcgaacacgaaatcgatcagaagtcttacatcttgcaaaagcataccatttccaagcaatctattgcttctttggttgaaggtggttgtttgttgttgccaattatcaaccaggacatcacctctaaagaacgtaaggacaagaatcagttctccaaggattggaagcaaatcttcgaaggttccaaagaattcagattgcatccagaattcgccgtttcttacagaactccaattgaaggttacccagtccaaaaaagatacggtagattgcaattcgtttgcgcttttaactgcgaaatcatcccacaaaatggtgagttcatcaacttgaagaagcagatcgagaacttcaacgacgaagatgctcaaaaagaagccgtcgaagagttcaacaaaaaggttaaccatgccttgtccgacaaagaatacgttgttattggtatcgacagaggcttgaagcaattagctactttgtgtgttttggacaagaggggtaagattttgggtgactttgaaatctacaaaaaagagttcgtcagagccgaaaagagatctgaatctcattgggaacatactcaagctgaaaccagacatatcttggacttgtctaacttgagagttgaaactaccattgagggcaaaaaggtgttggttgatcaatctttgacactggtcaagaagaacagagatactccagatgaagaagctaccgaagaaaacaagcagaagattaagttgaagcagctgtcctacattagaaagttgcaacacaagatgcagaccaatgaacaagatgtcttggacctgatcaacaacgaaccatctgatgaagaattcaaaaagaggatcgagggcttgatttcttcattcggtgaaggtcaaaagtacgctgatttgcctattaacaccatgagggaaatgatctctgacttgcaaggtgttattgccagaggaaacaatcagactgagaaaaacaagatcatcgaattggatgctgccgacaatttgaaacaaggtatcgttgctaacatgatcggtatcgttaactacattttcgccaagtactcctacaaggcctacatttctttagaagatttgtccagagcttacggtggtgcaaaatctggttatgatggtagatatttgccatccacctctcaagatgaggatgttgactttaaagaacagcagaatcaaatgttggctggcttgggtacttaccaattttttgaaatgcagctgctgaaaaagctgcagaagatccaatctgataacaccgttttgagatttgttccagcttttagatccgccgataactacagaaatatcttgagattggaagagactaagtacaagtctaagccattcggtgttgttcatttcatcgatccaaagttcacatctaagaagtgtccagtttgctctaagactaacgtttacagagataaggatgacatcctggtctgtaaagaatgtggttttaggtccgactcacagttgaaagaaagggaaaacaacatccactacatccacaatggtgatgataatggtgcttaccatattgccttgaagtccgtcgaaaacttgattcagatgaagtaa

SEQ ID NO: 6 - DNA, 3696 bp, synthetic construct
  misc_feature 1..3696: note = BEC10 NT Sequence (Yeast codon optimized)
  source 1..3696: mol_type = other DNA
atgaagtccttcgaaaactcctgccaaatttctaagactttgagattcggtgccactttgaaagaggataagaaaaagtgcaagtcccacttggaattgcaagaattcgttgacatttcctacaagaccttgaagtcatctgctaccattgctgaatccttgaacgaaatcgaattggtcaaaaagtgcgaaaggtgctactccgaaattatcaagttccatgaagcttggggtcaaatctactgtagaactaaccaaattgccgtctacaaggactggtatagacaattggctagaaaggccagattcgatgttggtgatcaaaactctcaactgatcaccttgtcatccttatcttctaagcacaacgtttaccagggtttgaagagatctcaacatattaccaactactggaaggacaacattgccagacaaaagtctttcctgaaggatttctctcaacaattgaagcagtacaagagagctttggaaaattctgataaggctcataccaagccaaacctgattaacttcaacaagaccttctccattttggccaacttggttaacgaaattgtcatcccattgtccaacggtgctatttcttttccaaacatctccaagttggaagatggtgaagaatccagacatttgattgaattcgctctgaacgattactccgatttggttggttctattggtgaattgaaggatgctattgctaccaatggtggttatactccatttgctaaggttaccttgaaccattacactgctgaacaaaagccacacgttttcaagaacgatattgatgccaagatccgtgagttgaagttgattgagttggtcgaaaagttgaagaacaagacgtccaagcaaatcgaagagtacttttccaagttcgacaagttcaagatctacgatgatagaaacatctccgttatcattagaacccaatgctttaagtacaagcccattccatttttggtcaagcacgaattggctaagtatatcgctgaagatgaagatgccgttttgaaggttttggatgcaattggtgctactagatctccagctcatgattacgctcataatgaagatgtttttgacttgaatcactacccaatcaaggttgcttttgattacgcatgggaacaattggctaacggtgtctacactactgttactttcccaaaagaacagtgcgagaagtacttgaaggatgtttttgattgcgaagtctccaaagaaccagtttttaagttctacgccgacctgttgtacatcagaaagaatttggctgttttggagcacaagaacaacctgccatctaatcaagaggaattcatctgcaagattaacaacaccttcgagaacatcgttctgccatacaagattaaagagttcgaaacctacaagaaggatatcttggcctggattaacgatggtagaggtcacgaaaagtacaccgatgctaaacaacagttgggttttattagaggtggtctgaaaggtagaatcaaggctcaaaagatgttcagaaaagacaagtacggtaagatcaagtcctactacgaaaacccatacactaagttgaccaacgaattcaagcaaatctcttctacctacggtaaaaccttcgctgaattgagagacaagttcaaagaaaagaacaacatcaccaagatcacccatttcggtattatcatcgaagataacaacaaagacagatacttgttggccaacggtttgcaacacgaacaaatcaaccatgtcgaagccattttgggtaagttgaacacctcatccgaattcatcacctaccaagttaagtctttgacctctaagaccctgatcaagctgattaagaatcataccaccaagaagggtgcaatttctccatatgctgatttccatacttctaagatccatgttgattggaccaagatcaagaaagaatgggacaactacaagagagaacaagtcttgttgcaatacgttaaggattgcttgaccgattctaccatggctaagaatcaaaattgggctgaatttggttggaacttcgagaagtgtaactcctacgaagatatcgaacacgaaatcgatcagaagtcttacatcttgcaaaagcataccatttccaagcaatctattgcttctttggttgaaggtggttgtttgttgttgccaattatcaaccaggacatcacctctcaaggtcgtaaggacaagaatcagttctccaaggattggaagcaaatcttcgaaggttccaaagaattcagattgcatccagaattcgccgtttcttacagaactccaattaaggactacccaaaggataaaagatacggtagattgcaattcgtttgcgcttttaactgcgaaatcatcccacaaaatggtgagttcatcaacttgaagaagcagatcgagaacttcaacgacgaagatgctcaaaaagaagccgtcgaagagttcaacaaaaaggttaaccatgccttgttgggtaaagaatacgttgttattggtatcgacagaggcttgaagcaattagctactttgtgtgttttggacaagaggggtaagattttgggtgactttgaaatctacaaaaaagagttcgtcagagccgaaaagagatctaagaattactggaagcacaccttggctgaaaccagacatatcttggacttgtctaacttgagagttgaaactaccattgaggataataaggtgttggttgatcaatctttgacactggtcaagaagaacagagatactccagatgaagaagctaccgaagaaaacaagcagaagattaagttgaagcagctgtcctacattagaaagttgcaacacaagatgcagaccaatgaacaagatgtcttggacctgatcaacaacgaaccatctgatgaagaattcaaaaagaggatcgagggcttgatttcttcattcggtgaaggtcaaaagtacgctgatttgcctattaacaccatgagggaaatgatctctgacttgcaaggtgttattgccagaggaaacaatcagactgagaaaaacaagatcatcgaattggatgctgccgacaatttgaaacaaggtatcgttgctaacatgatcggtatcgttaactacattttcgccaagtactcctacaaggcctacatttctttagaagatttgtccagagcttacggtggtgcaaaatctggttatgatggtagatatttgccatccacctctcaagatgaggatgttgactttaaagaacagcagaatcaaatgttggctggcttgggtacttaccaattttttgaaatgcagctgctgaaaaagctgcagaagatccaatctgataacaccgttttgagatttgttccagcttttagatccgccgataactacagaaatatcatcaagttggaagagactaagtacaagtctaagccattcggtgttgttcatttcatcgatccaaagttcacatctaagaagtgtccagtttgctctaagactaacgtttacagagataaggatgacatcctggtctgtaaagaatgtggttttaggtccgactcacagttgaaagaaagggaaaacaacatccactacatccacaatggtgatgataatggtgcttaccatattgccttgaagtccgtcgaaaacttgattcagatgaagtaa

SEQ ID NO: 7 - DNA, 3696 bp, synthetic construct
  misc_feature 1..3696: note = BEC10 NT Sequence (E. coli codon optimized)
  source 1..3696: mol_type = other DNA
atgaaaagctttgaaaacagctgccagattagcaaaaccctgcgttttggtgcaaccctgaaagaggataaaaagaaatgtaaaagccacctggaactgcaagaatttgtggatattagctacaagaccctgaaaagcagcgcaaccattgcagaaagcctgaatgaaattgagctggtgaaaaaatgcgaacgctgctatagcgaaatcatcaaatttcatgaagcctggggtcagatttattgtcgtaccaatcagattgccgtgtacaaagattggtatcgtcagctggcacgtaaagcacgttttgatgttggtgatcagaatagccagctgattaccctgagcagcctgagtagcaaacataatgtttatcagggtctgaaacgcagccagcatattaccaattattggaaagataacattgcccgtcagaaaagcttcctgaaagattttagccagcagctgaaacagtataaacgtgcactggaaaatagcgataaagcacataccaaaccgaacctgatcaacttcaataaaacctttagcattctggccaacctggtgaacgaaattgttattccgctgagcaatggtgcaattagctttccgaatatcagcaaactggaagatggtgaagaaagccgtcatctgattgaatttgccctgaatgattatagcgatctggttggtagcattggcgaactgaaagatgcaattgccaccaatggtggttataccccgtttgcaaaagttaccctgaaccattataccgcagaacagaaaccgcatgtgttcaaaaatgatatcgatgccaaaatccgtgagctgaaactgattgaactggttgagaaactgaaaaacaaaaccagcaagcagatcgaagagtacttcagcaaattcgacaagttcaaaatctatgatgatcgcaacatcagcgtgattattcgtacccagtgctttaaatacaaaccgattccgtttctggtgaaacatgaactggccaaatatatcgccgaagatgaagatgcagttctgaaagttctggatgccattggtgcgacccgtagtccggcacatgattatgcacataatgaagatgtgttcgatctgaaccactatccgattaaagtggcatttgattatgcctgggaacagctggcaaatggtgtgtataccaccgtgacctttccgaaagaacagtgtgaaaaatatctgaaggatgtgtttgattgcgaggttagcaaagaaccggtgtttaaattctatgccgatctgctgtatatccgcaaaaatctggccgttctggaacataaaaacaatctgccgagcaaccaagaagagttcatttgcaaaatcaacaacaccttcgaaaacatcgtgctgccgtataaaatcaaagagttcgaaacctacaaaaaagacatcctggcctggattaatgatggtcgtggtcatgagaaatataccgatgcaaaacagcagctgggttttattcgtggtggtctgaaaggtcgtattaaagcccagaaaatgttccgcaaagataagtacggtaagatcaaaagctattatgagaacccgtataccaaactgaccaacgaatttaagcagatcagcagcacctatggcaaaacctttgccgaactgcgtgataagtttaaagagaagaacaacatcaccaaaatcacccactttggcatcatcatcgaggataataacaaagatcgttatctgctggccaatggtctgcagcatgagcagattaatcatgttgaagcaattctgggcaaactgaataccagcagcgaatttatcacctatcaggttaaaagcctgaccagtaaaaccctgattaagctgattaaaaaccataccaccaaaaagggtgcgattagcccgtatgcagattttcataccagcaaaattcatgtggactggacgaaaatcaaaaaagagtgggataactataagcgcgaacaggttctgctgcagtatgttaaagattgtctgaccgatagcaccatggccaaaaatcagaattgggcagaatttggctggaactttgaaaaatgcaacagctatgaagatatcgagcacgagattgaccagaaaagttatatcctgcagaaacacaccatctccaaacagagcattgcaagcctggttgaaggtggttgtctgctgctgccgattattaaccaggatattacctcacagggtcgcaaagacaaaaaccagtttagtaaagattggaagcagatctttgaaggcagcaaagaatttcgtctgcatccggaatttgcagttagctatcgtaccccgatcaaagattatccgaaagataaacgttatggtcgcctgcagtttgtttgtgcctttaactgtgaaatcattccgcagaatggcgaattcatcaatctgaaaaagcagattgagaacttcaacgatgaggatgcacagaaagaagccgttgaagaattcaacaaaaaagtgaatcatgccctgctgggcaaagaatatgttgtgattggtattgatcgtggcctgaaacaactggcaaccctgtgtgttctggataaacgtggtaaaatcctgggcgattttgagatctacaagaaagaattcgttcgtgccgaaaaacgcagcaaaaactattggaaacacacactggcagaaacccgtcatattctggatctgagcaatctgcgtgttgaaaccacaatcgaagataacaaagtgctggttgatcagagtctgaccctggttaaaaagaatcgtgatacaccggatgaagaagccaccgaagaaaataaacagaagatcaaactgaagcagctgagctatattcgtaaactgcagcataaaatgcagaccaatgaacaggatgttctggacctgattaataacgaaccgagcgacgaagaatttaagaaacgtattgaaggtctgattagcagctttggtgaaggtcagaaatatgcggatctgcctattaataccatgcgcgaaatgattagtgatctgcagggtgttattgcccgtggtaataatcagacagagaaaaacaagatcatcgaactggatgcagccgataatctgaaacagggtattgttgcaaacatgattggcatcgtgaactacatctttgccaaatacagctacaaagcctatatcagcctggaagatctgagccgtgcatatggtggtgcaaaaagcggttatgatggacgctatctgccgtcaaccagccaggacgaagatgtggattttaaagaacagcagaatcagatgctggcaggtctgggtacatatcagttttttgaaatgcagctgctgaagaagctgcagaaaattcagagcgataataccgttctgcgctttgttccggcatttcgtagcgcagataactatcgcaatattatcaagctggaagaaaccaaatacaaaagcaaaccgtttggcgtggtgcactttattgatccgaaatttacgagcaaaaaatgtccggtttgcagcaaaaccaatgtgtatcgtgataaagatgacattctggtgtgtaaagaatgcggttttcgtagtgatagtcagctgaaagaacgcgaaaacaacatccactatattcataatggtgatgacaacggtgcctatcatattgcactgaaaagcgtggaaaatctgatccagatgaaataa

SEQ ID NO: 8 - DNA, 1191 bp, synthetic construct
  misc_feature 1..1191: note = araC-ParaBAD inducible promotor system
  source 1..1191: mol_type = other DNA
tatggagaaacagtagagagttgcgataaaaagcgtcaggtaggatccgctaatcttatggataaaaatgctatggcatagcaaagtgtgacgccgtgcaaataatcaatgtggacttttctgccgtgattatagacacttttgttacgcgtttttgtcatggctttggtcccgctttgttacagaatgcttttaataagcggggttaccggtttggttagcgagaagagccagtaaaagacgcagtgacggcaatgtctgatgcaatatggacaattggtttcttctctgaatggcgggagtatgaaaagtatggctgaagcgcaaaatgatcccctgctgccgggatactcgtttaatgcccatctggtggcgggtttaacgccgattgaggccaacggttatctcgatttttttatcgaccgaccgctgggaatgaaaggttatattctcaatctcaccattcgcggtcagggggtggtgaaaaatcagggacgagaatttgtttgccgaccgggtgatattttgctgttcccgccaggagagattcatcactacggtcgtcatccggaggctcgcgaatggtatcaccagtgggtttactttcgtccgcgcgcctactggcatgaatggcttaactggccgtcaatatttgccaatacggggttctttcgcccggatgaagcgcaccagccgcatttcagcgacctgtttgggcaaatcattaacgccgggcaaggggaagggcgctattcggagctgctggcgataaatctgcttgagcaattgttactgcggcgcatggaagcgattaacgagtcgctccatccaccgatggataatcgggtacgcgaggcttgtcagtacatcagcgatcacctggcagacagcaattttgatatcgccagcgtcgcacagcatgtttgcttgtcgccgtcgcgtctgtcacatcttttccgccagcagttagggattagcgtcttaagctggcgcgaggaccaacgtatcagccaggcgaagctgcttttgagcaccacccggatgcctatcgccaccgtcggtcgcaatgttggttttgacgatcaactctatttctcgcgggtatttaaaaaatgcaccggggccagcccgagcgagttccgtgccggttgtgaagaaaaagtgaatgatgtagccgtcaagttgtcataa

SEQ ID NO: 9 - DNA, 177 bp, synthetic construct
  misc_feature 1..177: note = fdT expression terminator
  source 1..177: mol_type = other DNA
aattttctgtatgaggttttgctaaacaactttcaacagtttcagcggagtgagaatagaaaggaacaactaaaggaattgcgaataataattttttcacgttgaaaatctccaaaaaaaaaggctccaaaaggagcctttaattgtatcggtttatcagcttgctttcgaggtgaa

SEQ ID NO: 10 - DNA, 10026 bp, synthetic construct
  misc_feature 1..10026: note = Nucleotide sequence of the CRISPR/BEC10-Ec vector system
  source 1..10026: mol_type = other DNA
ctaccggcgcggcagcgtgacccgtgtcggcggctccaacggctcgccatcgtccagaaaacacggctcatcgggcatcggcaggcgctgctgcccgcgccgttcccattcctccgtttcggtcaaggctggcaggtctggttccatgcccggaatgccgggctggctgggcggctcctcgccggggccggtcggtagttgctgctcgcccggatacagggtcgggatgcggcgcaggtcgccatgccccaacagcgattcgtcctggtcgtcgtgatcaaccaccacggcggcactgaacaccgacaggcgcaactggtcgcggggctggccccacgccacgcggtcattgaccacgtaggccgacacggtgccggggccgttgagcttcacgacggagatccagcgctcggccaccaagtccttgactgcgtattggaccgtccgcaaagaacgtccgatgagcttggaaagtgtcttttggctgaccaccacggcgttctggtggcccatctgcgccacgaggtgatgcagcagcattgccgccgtgggtttcctcgcaataagcccggcccacgcctcatgcgctttgcgttccgtttgcacccagtgaccgggcttgttcttggcttgaatgccgatttctctggactgcgtggccatgcttatctccatgcggtagggtgccgcacggttgcggcaccatgcgcaatcagctgcaacttttcggcagcgcgacaacaattatgcgttgcgtaaaagtggcagtcaattacagattttctttaacctacgcaatgagctattgcggggggtgccgcaatgagctgttgcgtaccccccttttttaagttgttgatttttaagtctttcgcatttcgccctatatctagttctttggtgcccaaagaagggcacccctgcggggttcccccacgccttcggcgcggctccccctccggcaaaaagtggcccctccggggcttgttgatcgactgcgcggccttcggccttgcccaaggtggcgctgcccccttggaacccccgcactcgccgccgtgaggctcggggggcaggcgggcgggcttcgccttcgactgcccccactcgcataggcttgggtcgttccaggcgcgtcaaggccaagccgctgcgcggtcgctgcgcgagccttgacccgccttccacttggtgtccaaccggcaagcgaagcgcgcaggccgcaggccggaggcttttccccagagaaaattaaaaaaattgatggggcaaggccgcaggccgcgcagttggagccggtgggtatgtggtcgaaggctgggtagccggtgggcaatccctgtggtcaagctcgtgggcaggcgcagcctgtccatcagcttgtccagcagggttgtccacgggccgagcgaagcgagccagccggtggccgctcgcggccatcgtccacatatccacgggctggcaagggagcgcagcgaccgcgcagggcgaagcccggagagcaagcccgtagggcgccgcagccgccgtaggcggtcacgactttgcgaagcaaagtctagtgagtatactcaagcattgagtggcccgccggaggcaccgccttgcgctgcccccgtcgagccggttggacaccaaaagggaggggcaggcatggcggcatacgcgatcatgcgatgcaagaagctggcgaaaatgggcaacgtggcggccagtctcaagcacgcctaccgcgagcgcgagacgcccaacgctgacgccagcaggacgccagagaacgagcactgggcggccagcagcaccgatgaagcgatgggccgactgcgcgagttgctgccagagaagcggcgcaaggacgctgtgttggcggtcgagtacgtcatgacggccagcccggaatggtggaagtcggccagccaagaacagcaggcggcgttcttcgagaaggcgcacaagtggctggcggacaagtacggggcggatcgcatcgtgacggccagcatccaccgtgacgaaaccagcccgcacatgaccgcgttcgtggtgccgctgacgcaggacggcaggctgtcggccaaggagttcatcggcaacaaagcgcagatgacccgcgaccagaccacgtttgcggccgctgtggccgatctagggctgcaacggggcatcgagggcagcaaggcacgtcacacgcgcattcaggcgttctacgaggccctggagcggccaccagtgggccacgtcaccatcagcccgcaagcggtcgagccacgcgcctatgcaccgcagggattggccgaaaagctgggaatctcaaagcgcgttgagacgccggaagccgtggccgaccggctgacaaaagcggttcggcaggggtatgagcctgccctacaggccgccgcaggagcgcgtgagatgcgcaagaaggccgatcaagcccaagagacggcccgagaccttcgggagcgcctgaagcccgttctggacgccctggggccgttgaatcgggatatgcaggccaaggccgccgcgatcatcaaggccgtgggcgaaaagctgctgacggaacagcgggaagtccagcgccagaaacaggcccagcgccagcaggaacgcgggcgcgcacatttccccgaaaagtgccacctgcgaaccccagagtcccgctcagaagaactcgtcaagaaggcgatagaaggcgatgcgctgcgaatcgggagcggcgataccgtaaagcacgaggaagcggtcagcccattcgccgccaagctcttcagcaatatcacgggtagccaacgctatgtcctgatagcggtccgccacacccagccggccacagtcgatgaatccagaaaagcggccattttccaccatgatattcggcaagcaggcatcgccatgggtcacgacgagatcctcgccgtcgggcatccgcgccttgagcctggcgaacagttcggctggcgcgagcccctgatgctcttcgtccagatcatcctgatcgacaagaccggcttccatccgagtacgtgctcgctcgatgcgatgtttcgcttggtggtcgaatgggcaggtagccggatcaagcgtatgcagccgccgcattgcatcagccatgatggatactttctcggcaggagcaaggtgagatgacaggagatcctgccccggcacttcgcccaatagcagccagtcccttcccgcttcagtgacaacgtcgagcacagctgcgcaaggaacgcccgtcgtggccagccacgatagccgcgctgcctcgtcttggagttcattcagggcaccggacaggtcggtcttgacaaaaagaaccgggcgcccctgcgctgacagccggaacacggcggcatcagagcagccgattgtctgttgtgcccagtcatagccgaatagcctctccacccaagcggccggagaacctgcgtgcaatccatcttgttcaatcatgcgaaacgatcctcatcctgtctcttgatcagatcttgatcccctgcgccatcagatccttggcggcaagaaagccatccagtttactttgcagggcttcccaaccttaccagagggcgccccagctggcaattccggttcgcttgctgtccataaaaccgcccagtctagctatcgccatgtaagcccactgcaagctacctgctttctctttgcgcttgcgttttcccttgtccagatagcccagtagctgacattcatccggggtcagcaccgtttctgcggactggctttctacgtgttccgcttcctttagcagcccttgcgccctgagtgcttgcggcagcgtgaagctagctgcataatgtgcctgtcaaatggacgaagcagggattctgcaaaccctatgctactccgtcaagccgtcaattgtctgattcgttaccaattatgacaacttgacggctacatcattcactttttcttcacaaccggcacggaactcgctcgggctggccccggtgcattttttaaatacccgcgagaaatagagttgatcgtcaaaaccaacattgcgaccgacggtggcgataggcatccgggtggtgctcaaaagcagcttcgcctggctgatacgttggtcctcgcgccagcttaagacgctaatccctaactgctggcggaaaagatgtgacagacgcgacggcgacaagcaaacatgctgtgcgacgctggcgatatcaaaattgctgtctgccaggtgatcgctgatgtactgacaagcctcgcgtacccgattatccatcggtggatggagcgactcgttaatcgcttccatgcgccgcagtaacaattgctcaagcagatttatcgccagcagctccgaatagcgcccttccccttgcccggcgttaatgatttgcccaaacaggtcgctgaaatgcggctggtgcgcttcatccgggcgaaagaaccccgtattggcaaatattgacggccagttaagccattcatgccagtaggcgcgcggacgaaagtaaacccactggtgataccattcgcgagcctccggatgacgaccgtagtgatgaatctctcctggcgggaacagcaaaatatcacccggtcggcaaacaaattctcgtccctgatttttcaccaccccctgaccgcgaatggtgagattgagaatataacctttcattcccagcggtcggtcgataaaaaaatcgagataaccgttggcctcaatcggcgttaaacccgccaccagatgggcattaaacgagtatcccggcagcaggggatcattttgcgcttcagccatacttttcatactcccgccattcagagaagaaaccaattgtccatattgcatcagacattgccgtcactgcgtcttttactggctcttctcgctaaccaaaccggtaaccccgcttattaaaagcattctgtaacaaagcgggaccaaagccatgacaaaaacgcgtaacaaaagtgtctataatcacggcagaaaagtccacattgattatttgcacggcgtcacactttgctatgccatagcatttttatccataagattagcggatcctacctgacgctttttatcgcaactctctactgtttctccatacccgttttttggtaccgggccccccctcgagtttattttaggaggcaaaaatgaaaagctttgaaaacagctgccagattagcaaaaccctgcgttttggtgcaaccctgaaagaggataaaaagaaatgtaaaagccacctggaactgcaagaatttgtggatattagctacaagaccctgaaaagcagcgcaaccattgcagaaagcctgaatgaaattgagctggtgaaaaaatgcgaacgctgctatagcgaaatcatcaaatttcatgaagcctggggtcagatttattgtcgtaccaatcagattgccgtgtacaaagattggtatcgtcagctggcacgtaaagcacgttttgatgttggtgatcagaatagccagctgattaccctgagcagcctgagtagcaaacataatgtttatcagggtctgaaacgcagccagcatattaccaattattggaaagataacattgcccgtcagaaaagcttcctgaaagattttagccagcagctgaaacagtataaacgtgcactggaaaatagcgataaagcacataccaaaccgaacctgatcaacttcaataaaacctttagcattctggccaacctggtgaacgaaattgttattccgctgagcaatggtgcaattagctttccgaatatcagcaaactggaagatggtgaagaaagccgtcatctgattgaatttgccctgaatgattatagcgatctggttggtagcattggcgaactgaaagatgcaattgccaccaatggtggttataccccgtttgcaaaagttaccctgaaccattataccgcagaacagaaaccgcatgtgttcaaaaatgatatcgatgccaaaatccgtgagctgaaactgattgaactggttgagaaactgaaaaacaaaaccagcaagcagatcgaagagtacttcagcaaattcgacaagttcaaaatctatgatgatcgcaacatcagcgtgattattcgtacccagtgctttaaatacaaaccgattccgtttctggtgaaacatgaactggccaaatatatcgccgaagatgaagatgcagttctgaaagttctggatgccattggtgcgacccgtagtccggcacatgattatgcacataatgaagatgtgttcgatctgaaccactatccgattaaagtggcatttgattatgcctgggaacagctggcaaatggtgtgtataccaccgtgacctttccgaaagaacagtgtgaaaaatatctgaaggatgtgtttgattgcgaggttagcaaagaaccggtgtttaaattctatgccgatctgctgtatatccgcaaaaatctggccgttctggaacataaaaacaatctgccgagcaaccaagaagagttcatttgcaaaatcaacaacaccttcgaaaacatcgtgctgccgtataaaatcaaagagttcgaaacctacaaaaaagacatcctggcctggattaatgatggtcgtggtcatgagaaatataccgatgcaaaacagcagctgggttttattcgtggtggtctgaaaggtcgtattaaagcccagaaaatgttccgcaaagataagtacggtaagatcaaaagctattatgagaacccgtataccaaactgaccaacgaatttaagcagatcagcagcacctatggcaaaacctttgccgaactgcgtgataagtttaaagagaagaacaacatcaccaaaatcacccactttggcatcatcatcgaggataataacaaagatcgttatctgctggccaatggtctgcagcatgagcagattaatcatgttgaagcaattctgggcaaactgaataccagcagcgaatttatcacctatcaggttaaaagcctgaccagtaaaaccctgattaagctgattaaaaaccataccaccaaaaagggtgcgattagcccgtatgcagattttcataccagcaaaattcatgtggactggacgaaaatcaaaaaagagtgggataactataagcgcgaacaggttctgctgcagtatgttaaagattgtctgaccgatagcaccatggccaaaaatcagaattgggcagaatttggctggaactttgaaaaatgcaacagctatgaagatatcgagcacgagattgaccagaaaagttatatcctgcagaaacacaccatctccaaacagagcattgcaagcctggttgaaggtggttgtctgctgctgccgattattaaccaggatattacctcacagggtcgcaaagacaaaaaccagtttagtaaagattggaagcagatctttgaaggcagcaaagaatttcgtctgcatccggaatttgcagttagctatcgtaccccgatcaaagattatccgaaagataaacgttatggtcgcctgcagtttgtttgtgcctttaactgtgaaatcattccgcagaatggcgaattcatcaatctgaaaaagcagattgagaacttcaacgatgaggatgcacagaaagaagccgttgaagaattcaacaaaaaagtgaatcatgccctgctgggcaaagaatatgttgtgattggtattgatcgtggcctgaaacaactggcaaccctgtgtgttctggataaacgtggtaaaatcctgggcgattttgagatctacaagaaagaattcgttcgtgccgaaaaacgcagcaaaaactattggaaacacacactggcagaaacccgtcatattctggatctgagcaatctgcgtgttgaaaccacaatcgaagataacaaagtgctggttgatcagagtctgaccctggttaaaaagaatcgtgatacaccggatgaagaagccaccgaagaaaataaacagaagatcaaactgaagcagctgagctatattcgtaaactgcagcataaaatgcagaccaatgaacaggatgttctggacctgattaataacgaaccgagcgacgaagaatttaagaaacgtattgaaggtctgattagcagctttggtgaaggtcagaaatatgcggatctgcctattaataccatgcgcgaaatgattagtgatctgcagggtgttattgcccgtggtaataatcagacagagaaaaacaagatcatcgaactggatgcagccgataatctgaaacagggtattgttgcaaacatgattggcatcgtgaactacatctttgccaaatacagctacaaagcctatatcagcctggaagatctgagccgtgcatatggtggtgcaaaaagcggttatgatggacgctatctgccgtcaaccagccaggacgaagatgtggattttaaagaacagcagaatcagatgctggcaggtctgggtacatatcagttttttgaaatgcagctgctgaagaagctgcagaaaattcagagcgataataccgttctgcgctttgttccggcatttcgtagcgcagataactatcgcaatattatcaagctggaagaaaccaaatacaaaagcaaaccgtttggcgtggtgcactttattgatccgaaatttacgagcaaaaaatgtccggtttgcagcaaaaccaatgtgtatcgtgataaagatgacattctggtgtgtaaagaatgcggttttcgtagtgatagtcagctgaaagaacgcgaaaacaacatccactatattcataatggtgatgacaacggtgcctatcatattgcactgaaaagcgtggaaaatctgatccagatgaaataatggtctagaggtcgaaattcaaattgtgagcggataacaatttgaattttctgtatgaggttttgctaaacaactttcaacagtttcagcggagtgagaatagaaaggaacaactaaaggaattgcgaataataattttttcacgttgaaaatctccaaaaaaaaaggctccaaaaggagcctttaattgtatcggtttatcagcttgctttcgaggtgaatttcgaccctctagcgaaaatgcaagagcaaagacgaaaacatgccacacatgaggaataccgattctctcattaacatattcaggccagttatctgggcttaaaagcagaagtccaacccagataacgatcatatacatggttctctccagaggttcattactgaacactcgtccgagaataacgagtggatcccctccaattcgccctatagtgagtcgtattacgcgcgctcactggccgtcgttttacaacgtcgtgactgggaaaaccctggcgttacccaacttaatcgccttgcagcacatccccctttcgccagctggcgtaatagcgaagaggcccgcaccgatcgcccttcccaacagttgcgcagcctgaatggcgaatggaaattgtaagcgttaatattttgttaaaattcgcgttaaatttttgttaaatcagctcattttttaaccaataggccgactgcgatgagtggcagggcggggcgtaatttttttaaggcagttattggtgcccttaaacgcctggtgctacgcctgaataagtgataataagcggatgaatggcagaaattcgaaagcaaattcgacccggtcgtcggttcagggcagggtcgttaaatagccgcttatgtctattgctggtttaccggtttattgactaccggaagcagtgtgaccgtgtgcttctcaaatgcctgaggccagtttgctcaggctctccccgtggaggtaataattgacgatatgatcatttattctgcctcccagagcctgataaaaacggtgaatccgttagcgaggtgccgccggcttccattcaggtcgaggtggcccggctccatgcaccgcgacgcaacgcggggaggcagacaaggtatagggcggcgaggcggctacagccgatagtctggaacagcgcacttacgggttgctgcgcaacccaagtg

SEQ ID NO: 11 - DNA, 10225 bp, synthetic construct
  misc_feature 1..10225: note = Nucleotide sequence of the CRISPR/FnCpf1-Ec vector system
  source 1..10225: mol_type = other DNA
ctaccggcgcggcagcgtgacccgtgtcggcggctccaacggctcgccatcgtccagaaaacacggctcatcgggcatcggcaggcgctgctgcccgcgccgttcccattcctccgtttcggtcaaggctggcaggtctggttccatgcccggaatgccgggctggctgggcggctcctcgccggggccggtcggtagttgctgctcgcccggatacagggtcgggatgcggcgcaggtcgccatgccccaacagcgattcgtcctggtcgtcgtgatcaaccaccacggcggcactgaacaccgacaggcgcaactggtcgcggggctggccccacgccacgcggtcattgaccacgtaggccgacacggtgccggggccgttgagcttcacgacggagatccagcgctcggccaccaagtccttgactgcgtattggaccgtccgcaaagaacgtccgatgagcttggaaagtgtcttttggctgaccaccacggcgttctggtggcccatctgcgccacgaggtgatgcagcagcattgccgccgtgggtttcctcgcaataagcccggcccacgcctcatgcgctttgcgttccgtttgcacccagtgaccgggcttgttcttggcttgaatgccgatttctctggactgcgtggccatgcttatctccatgcggtagggtgccgcacggttgcggcaccatgcgcaatcagctgcaacttttcggcagcgcgacaacaattatgcgttgcgtaaaagtggcagtcaattacagattttctttaacctacgcaatgagctattgcggggggtgccgcaatgagctgttgcgtaccccccttttttaagttgttgatttttaagtctttcgcatttcgccctatatctagttctttggtgcccaaagaagggcacccctgcggggttcccccacgccttcggcgcggctccccctccggcaaaaagtggcccctccggggcttgttgatcgactgcgcggccttcggccttgcccaaggtggcgctgcccccttggaacccccgcactcgccgccgtgaggctcggggggcaggcgggcgggcttcgccttcgactgcccccactcgcataggcttgggtcgttccaggcgcgtcaaggccaagccgctgcgcggtcgctgcgcgagccttgacccgccttccacttggtgtccaaccggcaagcgaagcgcgcaggccgcaggccggaggcttttccccagagaaaattaaaaaaattgatggggcaaggccgcaggccgcgcagttggagccggtgggtatgtggtcgaaggctgggtagccggtgggcaatccctgtggtcaagctcgtgggcaggcgcagcctgtccatcagcttgtccagcagggttgtccacgggccgagcgaagcgagccagccggtggccgctcgcggccatcgtccacatatccacgggctggcaagggagcgcagcgaccgcgcagggcgaagcccggagagcaagcccgtagggcgccgcagccgccgtaggcggtcacgactttgcgaagcaaagtctagtgagtatactcaagcattgagtggcccgccggaggcaccgccttgcgctgcccccgtcgagccggttggacaccaaaagggaggggcaggcatggcggcatacgcgatcatgcgatgcaagaagctggcgaaaatgggcaacgtggcggccagtctcaagcacgcctaccgcgagcgcgagacgcccaacgctgacgccagcaggacgccagagaacgagcactgggcggccagcagcaccgatgaagcgatgggccgactgcgcgagttgctgccagagaagcggcgcaaggacgctgtgttggcggtcgagtacgtcatgacggccagcccggaatggtggaagtcggccagccaagaacagcaggcggcgttcttcgagaaggcgcacaagtggctggcggacaagtacggggcggatcgcatcgtgacggccagcatccaccgtgacgaaaccagcccgcacatgaccgcgttcgtggtgccgctgacgcaggacggcaggctgtcggccaaggagttcatcggcaacaaagcgcagatgacccgcgaccagaccacgtttgcggccgctgtggccgatctagggctgcaacggggcatcgagggcagcaaggcacgtcacacgcgcattcaggcgttctacgaggccctggagcggccaccagtgggccacgtcaccatcagcccgcaagcggtcgagccacgcgcctatgcaccgcagggattggccgaaaagctgggaatctcaaagcgcgttgagacgccggaagccgtggccgaccggctgacaaaagcggttcggcaggggtatgagcctgccctacaggccgccgcaggagcgcgtgagatgcgcaagaaggccgatcaagcccaagagacggcccgagaccttcgggagcgcctgaagcccgttctggacgccctggggccgttgaatcgggatatgcaggccaaggccgccgcgatcatcaaggccgtgggcgaaaagctgctgacggaacagcgggaagtccagcgccagaaacaggcccagcgccagcaggaacgcgggcgcgcacatttccccgaaaagtgccacctgcgaaccccagagtcccgctcagaagaactcgtcaagaaggcgatagaaggcgatgcgctgcgaatcgggagcggcgataccgtaaagcacgaggaagcggtcagcccattcgccgccaagctcttcagcaatatcacgggtagccaacgctatgtcctgatagcggtccgccacacccagccggccacagtcgatgaatccagaaaagcggccattttccaccatgatattcggcaagcaggcatcgccatgggtcacgacgagatcctcgccgtcgggcatccgcgccttgagcctggcgaacagttcggctggcgcgagcccctgatgctcttcgtccagatcatcctgatcgacaagaccggcttccatccgagtacgtgctcgctcgatgcgatgtttcgcttggtggtcgaatgggcaggtagccggatcaagcgtatgcagccgccgcattgcatcagccatgatggatactttctcggcaggagcaaggtgagatgacaggagatcctgccccggcacttcgcccaatagcagccagtcccttcccgcttcagtgacaacgtcgagcacagctgcgcaaggaacgcccgtcgtggccagccacgatagccgcgctgcctcgtcttggagttcattcagggcaccggacaggtcggtcttgacaaaaagaaccgggcgcccctgcgctgacagccggaacacggcggcatcagagcagccgattgtctgttgtgcccagtcatagccgaatagcctctccacccaagcggccggagaacctgcgtgcaatccatcttgttcaatcatgcgaaacgatcctcatcctgtctcttgatcagatcttgatcccctgcgccatcagatccttggcggcaagaaagccatccagtttactttgcagggcttcccaaccttaccagagggcgccccagctggcaattccggttcgcttgctgtccataaaaccgcccagtctagctatcgccatgtaagcccactgcaagctacctgctttctctttgcgcttgcgttttcccttgtccagatagcccagtagctgacattcatccggggtcagcaccgtttctgcggactggctttctacgtgttccgcttcctttagcagcccttgcgccctgagtgcttgcggcagcgtgaagctagctgcataatgtgcctgtcaaatggacgaagcagggattctgcaaaccctatgctactccgtcaagccgtcaattgtctgattcgttaccaattatgacaacttgacggctacatcattcactttttcttcacaaccggcacggaactcgctcgggctggccccggtgcattttttaaatacccgcgagaaatagagttgatcgtcaaaaccaacattgcgaccgacggtggcgataggcatccgggtggtgctcaaaagcagcttcgcctggctgatacgttggtcctcgcgccagcttaagacgctaatccctaactgctggcggaaaagatgtgacagacgcgacggcgacaagcaaacatgctgtgcgacgctggcgatatcaaaattgctgtctgccaggtgatcgctgatgtactgacaagcctcgcgtacccgattatccatcggtggatggagcgactcgttaatcgcttccatgcgccgcagtaacaattgctcaagcagatttatcgccagcagctccgaatagcgcccttccccttgcccggcgttaatgatttgcccaaacaggtcgctgaaatgcggctggtgcgcttcatccgggcgaaagaaccccgtattggcaaatattgacggccagttaagccattcatgccagtaggcgcgcggacgaaagtaaacccactggtgataccattcgcgagcctccggatgacgaccgtagtgatgaatctctcctggcgggaacagcaaaatatcacccggtcggcaaacaaattctcgtccctgatttttcaccaccccctgaccgcgaatggtgagattgagaatataacctttcattcccagcggtcggtcgataaaaaaatcgagataaccgttggcctcaatcggcgttaaacccgccaccagatgggcattaaacgagtatcccggcagcaggggatcattttgcgcttcagccatacttttcatactcccgccattcagagaagaaaccaattgtccatattgcatcagacattgccgtcactgcgtcttttactggctcttctcgctaaccaaaccggtaaccccgcttattaaaagcattctgtaacaaagcgggaccaaagccatgacaaaaacgcgtaacaaaagtgtctataatcacggcagaaaagtccacattgattatttgcacggcgtcacactttgctatgccatagcatttttatccataagattagcggatcctacctgacgctttttatcgcaactctctactgtttctccatacccgttttttggtaccgggccccccctcgagtttattttaggaggcaaaaatgtcaatttatcaagaatttgttaataaatatagtttaagtaaaactctaagatttgagttaatcccacagggtaaaacacttgaaaacataaaagcaagaggtttgattttagatgatgagaaaagagctaaagactacaaaaaggctaaacaaataattgataaatatcatcagttttttatagaggagatattaagttcggtttgtattagcgaagatttattacaaaactattctgatgtttattttaaacttaaaaagagtgatgatgataatctacaaaaagattttaaaagtgcaaaagatacgataaagaaacaaatatctgaatatataaaggactcagagaaatttaagaatttgtttaatcaaaaccttatcgatgctaaaaaagggcaagagtcagatttaattctatggctaaagcaatctaaggataatggtatagaactatttaaagccaatagtgatatcacagatatagatgaggcgttagaaataatcaaatcttttaaaggttggacaacttattttaagggttttcatgaaaatagaaaaaatgtttatagtagcaatgatattcctacatctattatttataggatagtagatgataatttgcctaaatttctagaaaataaagctaagtatgagagtttaaaagacaaagctccagaagctataaactatgaacaaattaaaaaagatttggcagaagagctaacctttgatattgactacaaaacatctgaagttaatcaaagagttttttcacttgatgaagtttttgagatagcaaactttaataattatctaaatcaaagtggtattactaaatttaatactattattggtggtaaatttgtaaatggtgaaaatacaaagagaaaaggtataaatgaatatataaatctatactcacagcaaataaatgataaaacactcaaaaaatataaaatgagtgttttatttaagcaaattttaagtgatacagaatctaaatcttttgtaattgataagttagaagatgatagtgatgtagttacaacgatgcaaagtttttatgagcaaatagcagcttttaaaacagtagaagaaaaatctattaaagaaacactatctttattatttgatgatttaaaagctcaaaaacttgatttgagtaaaatttattttaaaaatgataaatctcttactgatctatcacaacaagtttttgatgattatagtgttattggtacagcggtactagaatatataactcaacaaatagcacctaaaaatcttgataaccctagtaagaaagagcaagaattaatagccaaaaaaactgaaaaagcaaaatacttatctctagaaactataaagcttgccttagaagaatttaataagcatagagatatagataaacagtgtaggtttgaagaaatacttgcaaactttgcggctattccgatgatatttgatgaaatagctcaaaacaaagacaatttggcacagatatctatcaaatatcaaaatcaaggtaaaaaagacctacttcaagctagtgcggaagatgatgttaaagctatcaaggatcttttagatcaaactaataatctcttacataaactaaaaatatttcatattagtcagtcagaagataaggcaaatattttagacaaggatgagcatttttatctagtatttgaggagtgctactttgagctagcgaatatagtgcctctttataacaaaattagaaactatataactcaaaagccatatagtgatgagaaatttaagctcaattttgagaactcgactttggctaatggttgggataaaaataaagagcctgacaatacggcaattttatttatcaaagatgataaatattatctgggtgtgatgaataagaaaaataacaaaatatttgatgataaagctatcaaagaaaataaaggcgagggttataaaaaaattgtttataaacttttacctggcgcaaataaaatgttacctaaggttttcttttctgctaaatctataaaattttataatcctagtgaagatatacttagaataagaaatcattccacacatacaaaaaatggtagtcctcaaaaaggatatgaaaaatttgagtttaatattgaagattgccgaaaatttatagatttttataaacagtctataagtaagcatccggagtggaaagattttggatttagattttctgatactcaaagatataattctatagatgaattttatagagaagttgaaaatcaaggctacaaactaacttttgaaaatatatcagagagctatattgatagcgtagttaatcagggtaaattgtacctattccaaatctataataaagatttttcagcttatagcaaagggcgaccaaatctacatactttatattggaaagcgctgtttgatgagagaaatcttcaagatgtggtttataagctaaatggtgaggcagagcttttttatcgtaaacaatcaatacctaaaaaaatcactcacccagctaaagaggcaatagctaataaaaacaaagataatcctaaaaaagagagtgtttttgaatatgatttaatcaaagataaacgctttactgaagataagtttttctttcactgtcctattacaatcaattttaaatctagtggagctaataagtttaatgatgaaatcaatttattgctaaaagaaaaagcaaatgatgttcatatattaagtatagatagaggtgaaagacatttagcttactatactttggtagatggtaaaggcaatatcatcaaacaagatactttcaacatcattggtaatgatagaatgaaaacaaactaccatgataagcttgctgcaatagagaaagatagggattcagctaggaaagactggaaaaagataaataacatcaaagagatgaaagagggctatctatctcaggtagttcatgaaatagctaagctagttatagagtataatgctattgtggtttttgaggatttaaattttggatttaaaagagggcgtttcaaggtagagaagcaggtctatcaaaagttagaaaaaatgctaattgagaaactaaactatctagttttcaaagataatgagtttgataaaactgggggagtgcttagagcttatcagctaacagcaccttttgagacttttaaaaagatgggtaaacaaacaggtattatctactatgtaccagctggttttacttcaaaaatttgtcctgtaactggttttgtaaatcagttatatcctaagtatgaaagtgtcagcaaatctcaagagttctttagtaagtttgacaagatttgttataaccttgataagggctattttgagtttagttttgattataaaaactttggtgacaaggctgccaaaggcaagtggactatagctagctttgggagtagattgattaactttagaaattcagataaaaatcataattgggatactcgagaagtttatccaactaaagagttggagaaattgctaaaagattattctatcgaatatgggcatggcgaatgtatcaaagcagctatttgcggtgagagcgacaaaaagttttttgctaagctaactagtgtcctaaatactatcttacaaatgcgtaactcaaaaacaggtactgagttagattatctaatttcaccagtagcagatgtaaatggcaatttctttgattcgcgacaggcgccaaaaaatatgcctcaagatgctgatgccaatggtgcttatcatattgggctaaaaggtctgatgctactaggtaggatcaaaaataatcaagagggcaaaaaactcaatttggttatcaaaaatgaagagtattttgagttcgtgcagaataggaataactaaaggtcgaaattcaaattgtgagcggataacaatttgaattttctgtatgaggttttgctaaacaactttcaacagtttcagcggagtgagaatagaaaggaacaactaaaggaattgcgaataataattttttcacgttgaaaatctccaaaaaaaaaggctccaaaaggagcctttaattgtatcggtttatcagcttgctttcgaggtgaatttcgaccctctagcgaaaatgcaagagcaaagacgaaaacatgccacacatgaggaataccgattctctcattaacatattcaggccagttatctgggcttaaaagcagaagtccaacccagataacgatcatatacatggttctctccagaggttcattactgaacactcgtccgagaataacgagtggatcccctccaattcgccctatagtgagtcgtattacgcgcgctcactggccgtcgttttacaacgtcgtgactgggaaaaccctggcgttacccaacttaatcgccttgcagcacatccccctttcgccagctggcgtaatagcgaagaggcccgcaccgatcgcccttcccaacagttgcgcagcctgaatggcgaatggaaattgtaagcgttaatattttgttaaaattcgcgttaaatttttgttaaatcagctcattttttaaccaataggccgactgcgatgagtggcagggcggggcgtaatttttttaaggcagttattggtgcccttaaacgcctggtgctacgcctgaataagtgataataagcggatgaatggcagaaattcgaaagcaaattcgacccggtcgtcggttcagggcagggtcgttaaatagccgcttatgtctattgctggtttaccggtttattgactaccggaagcagtgtgaccgtgtgcttctcaaatgcctgaggccagtttgctcaggctctccccgtggaggtaataattgacgatatgatcatttattctgcctcccagagcctgataaaaacggtgaatccgttagcgaggtgccgccggcttccattcaggtcgaggtggcccggctccatgcaccgcgacgcaacgcggggaggcagacaaggtatagggcggcgaggcggctacagccgatagtctggaacagcgcacttacgggttgctgcgcaacccaagtg

SEQ ID NO: 12 - DNA, 165 bp, synthetic construct
  misc_feature 1..165: note = Nucleotide sequence of the PsacB RNA polymerase II promotor fromBacillus megaterium
  source 1..165: mol_type = other DNA
gcccatgcaacagaaactataaaaaatacagagaatgaaaagaaacagatagattttttagttctttaggcccgtagtctgcaaatccttttatgattttctatcaaacaaaagaggaaaatagaccagttgcaatccaaacgagagtctaatagaatgaggtcg

SEQ ID NO: 13 - DNA, 169 bp, synthetic construct
  misc_feature 1..169: note = Nucleotide sequence of the transcription T1 and T2 terminationregion of the E. coli rrnB gene
  source 1..169: mol_type = other DNA
tttgcctggcggcagtagcgcggtggtcccacctgaccccatgccgaactcagaagtgaaacgccgtagcgccgatggtagtgtggggtctccccatgcgagagtagggaactgccaggcatcaaataaaacgaaaggctcagtcgaaagactgggcctttcgttttat

SEQ ID NO: 14 - DNA, 19 bp, synthetic construct
  misc_feature 1..19: note = BEC family Stem-Loop sequence
  source 1..19: mol_type = other DNA
aatttctactgttgtagat

SEQ ID NO: 15 - DNA, 24 bp, synthetic construct
  misc_feature 1..24: note = Kanamycin target-specific 24 bps spacer sequence
  source 1..24: mol_type = other DNA
tcggcaggagcaaggtgagatgac

SEQ ID NO: 16 - DNA, 5039 bp, synthetic construct
  misc_feature 1..5039: note = Nucleotide sequence of the CRISPR/gRNA-Ec vector system
  source 1..5039: mol_type = other DNA
gacgaaagggcctcgtgatacgcctatttttataggttaatgtcatgataataatggtttcttagacgtcaggtggcacttttcggggaaatgtgcgcggaacccctatttgtttatttttctaaatacattcaaatatgtatccgctcatgagacaataaccctgataaatgcttcaataatattgaaaaaggaagagtatgagtattcaacatttccgtgtcgcccttattcccttttttgcggcattttgccttcctgtttttgctcacccagaaacgctggtgaaagtaaaagatgctgaagatcagttgggtgcacgagtgggttacatcgaactggatctcaacagcggtaagatccttgagagttttcgccccgaagaacgttttccaatgatgagcacttttaaagttctgctatgtggcgcggtattatcccgtattgacgccgggcaagagcaactcggtcgccgcatacactattctcagaatgacttggttgagtactcaccagtcacagaaaagcatcttacggatggcatgacagtaagagaattatgcagtgctgccataaccatgagtgataacactgcggccaacttacttctgacaacgatcggaggaccgaaggagctaaccgcttttttgcacaacatgggggatcatgtaactcgccttgatcgttgggaaccggagctgaatgaagccataccaaacgacgagcgtgacaccacgatgcctgtagcaatggcaacaacgttgcgcaaactattaactggcgaactacttactctagcttcccggcaacaattaatagactggatggaggcggataaagttgcaggaccacttctgcgctcggcccttccggctggctggtttattgctgataaatctggagccggtgagcgtgggtctcgcggtatcattgcagcactggggccagatggtaagccctcccgtatcgtagttatctacacgacggggagtcaggcaactatggatgaacgaaatagacagatcgctgagataggtgcctcactgattaagcattggtaactgtcagaccaagtttactcatatatactttagattgatttaaaacttcatttttaatttaaaaggatctaggtgaagatcctttttgataatctcatgaccaaaatcccttaacgtgagttttcgttccactgagcgtcagaccccgtagaaaagatcaaaggatcttcttgagatcctttttttctgcgcgtaatctgctgcttgcaaacaaaaaaaccaccgctaccagcggtggtttgtttgccggatcaagagctaccaactctttttccgaaggtaactggcttcagcagagcgcagataccaaatactgtccttctagtgtagccgtagttaggccaccacttcaagaactctgtagcaccgcctacatacctcgctctgctaatcctgttaccagtggctgctgccagtggcgataagtcgtgtcttaccgggttggactcaagacgatagttaccggataaggcgcagcggtcgggctgaacggggggttcgtgcacacagcccagcttggagcgaacgacctacaccgaactgagatacctacagcgtgagctatgagaaagcgccacgcttcccgaagggagaaaggcggacaggtatccggtaagcggcagggtcggaacaggagagcgcacgagggagcttccagggggaaacgcctggtatctttatagtcctgtcgggtttcgccacctctgacttgagcgtcgatttttgtgatgctcgtcaggggggcggagcctatggaaaaacgccagcaacgcggcctttttacggttcctggccttttgctggccttttgctcacatgttctttcctgcgttatcccctgattctgtggataaccgtattaccgcctttgagtgagctgataccgctcgccgcagccgaacgaccgagcgcagcgagtcagtgagcgaggaagcggaagagcgcccaatacgcaaaccgcctctccccgcgcgttggccgattcattaatgcagctggcacgacaggtttcccgactggaaagcgggcagtgagcgcaacgcaattaatgtgagttagctcactcattaggcaccccaggctttacactttatgcttccggctcgtatgttgtgtggaattgtgagcggataacaatttcacacaggaaacagctatgaccatgattacgccaagctcggaattaaccctcactaaagggaacaaaagctggagctctgcagcccatgcaacagaaactataaaaaatacagagaatgaaaagaaacagatagattttttagttctttaggcccgtagtctgcaaatccttttatgattttctatcaaacaaaagaggaaaatagaccagttgcaatccaaacgagagtctaatagaatgaggtcgaatttctactgttgtagattcggcaggagcaaggtgagatgacggccggcatggtcccagcctcctcgctggcgccggctgggcaacatgcttcggcatggcgaatgggactttttttttgcctggcggcagtagcgcggtggtcccacctgaccccatgccgaactcagaagtgaaacgccgtagcgccgatggtagtgtggggtctccccatgcgagagtagggaactgccaggcatcaaataaaacgaaaggctcagtcgaaagactgggcctttcgttttatggtacccaattcgccctatagtgagtcgtattacaattcactggccgtcgttttacaacgtcgtgactgggaaaaccctggcgttacccaacttaatcgccttgcagcacatccccctttcgccagctggcgtaatagcgaagaggcccgcaccgatcgcccttcccaacagttgcgcagcctgaaaggcaggccgggccgtggtggccacggcctctaggccagatccagcggcatctgggttagtcgagcgcgggccgcttcccatgtctcaccagggcgagcctgtttcgcgatctcagcatctgaaatcttcccggccttgcgcttcgctggggccttacccaccgccttggcgggcttcttcggtccaaaactgaacaacagatgtgtgaccttgcgcccggtctttcgctgcgcccactccacctgtagcgggctgtgctcgttgatctgcgtcacggctggatcaagcactcgcaacttgaagtccttgatcgagggataccggccttccagttgaaaccactttcgcagctggtcaatttctatttcgcgctggccgatgctgtcccattgcatgagcagctcgtaaagcctgatcgcgtgggtgctgtccatcttggccacgtcagccaaggcgtatttggtgaactgtttggtgagttccgtcaggtacggcagcatgtctttggtgaacctgagttctacacggccctcaccctcccggtagatgattgtttgcacccagccggtaatcatcacactcggtcttttccccttgccattgggctcttgggttaaccggacttcccgccgtttcaggcgcagggccgcttctttgagctggttgtaggaagattcgatagggacacccgccatcgtcgctatgtcctccgccgtcactgaatacatcacttcatcggtgacaggctcgctcctcttcacctggctaatacaggccagaacgatccgctgttcctgaacactgaggcgatacgcggcctcgaccagggcattgcttttgtaaaccattgggggtgaggccacgttcgacattccttgtgtataaggggacactgtatctgcgtcccacaatacaacaaatccgtccctttacaacaacaaatccgtcccttcttaacaacaaatccgtcccttaatggcaacaaatccgtccctttttaaactctacaggccacggattacgtggcctgtagacgtcctaaaaggtttaaaagggaaaaggaagaaaagggtggaaacgcaaaaaacgcaccactacgtggccccgttggggccgcatttgtgcccctgaaggggcgggggaggcgtctgggcaatccccgttttaccagtcccctatcgccgcctgagagggcgcaggaagcgagtaatcagggtatcgaggcggattcacccttggcgtccaaccagcggcaccagcggcgcctgagaggcctacagagcggttggacaccaaggggaggggctaagaccggtttatcagtcccctttccctcgtttctttccaacgcgatagcccagcaaggccgccaccgttgccaccgtcaccccagcaagcacagccagtggcgtgtaattggggtctgacgctcagtggaacgaaaactcacgttaagggattttggtcatgagattatcaaaaaggatcttcacctagatccttttaaattaaaaatgaagttttaaatcaatctaaagtatatatgagtaaacttggtctgacagttaccaatgcttaatcagtgaggcacctatctcagcgatctgtctatttcgttcatccatagttgcctgactccccgtcgtgtagataactacgatacgggagggcttaccatctggccccagtgctgcaatgataccgcgagatccacgctcaccggctccagatttatcagcaataaaccagccagccggaagggccgagcgcagaagtggtcctgcaactttatccgcctccatccagtctattaattgttgccgggaagctagagtaagtagttcgccagttaatagtttgcgcaacgttgttgccattgccgcctgatgcggtattttctccttacgcatctgtgcggtatttcacaccgcatatggtgcactctcagtacaatctgctctgatgccgcatagttaagccagccccgacacccgccaacacccgctgacgcgccctgacgggcttgtctgctcccggcatccgcttacagacaagctgtgaccgtctccgggagctgcatgtgtcagaggttttcaccgtcatcaccgaaacgcgcga

SEQ ID NO: 17 - DNA, 27 bp, synthetic construct
  misc_feature 1..27: note = SV40 nuclear localization signal (NLS)
  source 1..27: mol_type = other DNA
atggctcccaaaaagaaaaggaaggtg

SEQ ID NO: 18 - DNA, 548 bp, synthetic construct
  misc_feature 1..548: note = Nucleotide sequence of the p. pastoris HTX-Promotor
  source 1..548: mol_type = other DNA
tgatttgtttaggtaacttgaactggatgtattagtttggtgacaagcggatgtgggatatcagtgtgtttatatatacgtgatggggggaggactctcgtttcctatgataccttatggaatgggacagtacgcgctaatttgtctcgttctggatagactgctctgtttttcgttacatacgagtgggaagtgcgaacttttgtaccagagtgcgaaaaaagtggtggcaatcctgacgtttgtaccaagcgcgacggcacattattggtcagtttgtgcattttagtttttcttgaaaacatctcgaaacataacaactaggacaccaattctacagtgaaaaccattcagtggaatgtgaacccacataaatcttgcagcaataatacaacaatttatggctcctgcattctgattggctgagcgtttattgccatcgtgactgtccaatttaggacacaccctttcctcagaatatataaactggtgataattccttcgttctgagttccatctcatactcaaactatattaaaactacaaca

SEQ ID NO: 19 - DNA, 260 bp, synthetic construct
  misc_feature 1..260: note = Nucleotide sequence of the P. pastoris AOX1TT-Terminator
  source 1..260: mol_type = other DNA
tcaagaggatgtcagaatgccatttgcctgagagatgcaggcttcatttttgatacttttttatttgtaacctatatagtataggattttttttgtcattttgtttcttctcgtacgagcttgctcctgatcagcctatctcgcagcagatgaatatcttgtggtaggggtttgggaaaatcattcgagtttgatgtttttcttggtatttcccactcctcttcagagtacagaagattaagtgagaccttcgtttgtgc

SEQ ID NO: 20 - DNA, 810 bp, synthetic construct
  misc_feature 1..810: note = Nucleotide sequence of the kanMX6 marker gene
  source 1..810: mol_type = other DNA
atgggtaaggaaaagactcacgtttcgaggccgcgattaaattccaacatggatgctgatttatatgggtataaatgggctcgcgataatgtcgggcaatcaggtgcgacaatctatcgattgtatgggaagcccgatgcgccagagttgtttctgaaacatggcaaaggtagcgttgccaatgatgttacagatgagatggtcagactaaactggctgacggaatttatgcctcttccgaccatcaagcattttatccgtactcctgatgatgcatggttactcaccactgcgatccccggcaaaacagcattccaggtattagaagaatatcctgattcaggtgaaaatattgttgatgcgctggcagtgttcctgcgccggttgcattcgattcctgtttgtaattgtccttttaacagcgatcgcgtatttcgtctcgctcaggcgcaatcacgaatgaataacggtttggttgatgcgagtgattttgatgacgagcgtaatggctggcctgttgaacaagtctggaaagaaatgcataagcttttgccattctcaccggattcagtcgtcactcatggtgatttctcacttgataaccttatttttgacgaggggaaattaataggttgtattgatgttggacgagtcggaatcgcagaccgataccaggatcttgccatcctatggaactgcctcggtgagttttctccttcattacagaaacggctttttcaaaaatatggtattgataatcctgatatgaataaattgcagtttcatttgatgctcgatgagtttttctaa

SEQ ID NO: 21 - DNA, 624 bp, synthetic construct
  misc_feature 1..624: note = Nucleotide sequence of the bifunctional ILV5/synthetic Em72Promotor
  source 1..624: mol_type = other DNA
ggatccttcagtaatgtcttgtttcttttgttgcagtggtgagccattttgacttcgtgaaagtttctttagaatagttgtttccagaggccaaacattccacccgtagtaaagtgcaagcgtaggagcaccaagactggcataaatcaggtataagtgtcgagcactggcaggtgatcttctgaaagtttctactagcagataagatccagtagtcatgcatatggcaacaatgtaccgtgtggatctaagaacgcgtcctactaaccttcgcattcgttggtccagtttgttgttatcgatcaacgtgacaaggttgtcgattccgcgtaagcatgcatacccaaggacgcctgttgcaattccaagtgagccagttccaacaatctttgtaatattagagcacttcattgtgttgcgcttgaaagtaaaatgcgaacaaattaagagataatctcgaaaccgcgacttcaaacgccaatatgatgtgcggcacacaataagcgttcatatccgctgggtgactttctcgctttaaaaaattatccgaaaaaattttctagagtgttgttactttatacttccggctcgtataatacgacaaggtgtaaggaggactaaacc

SEQ ID NO: 22 - DNA, 156 bp, synthetic construct
  misc_feature 1..156: note = Nucleotide sequence of the pichia autonomously replicatingsequence 1 (PARS1)
  source 1..156: mol_type = other DNA
caattaatatttacttattttggtcaaccccaaataggttgatttcatacttggttcattcaaaaataagtagtcttttgagatctttcaatattataataaatatactataacagccgacttgtttcattttcgcgaatgttcccccagcttatc

SEQ ID NO: 23 - DNA, 24 bp, synthetic construct
  misc_feature 1..24: note = Ade2 target-specific 24 bps spacer sequence (BEC10)
  source 1..24: mol_type = other DNA
tcaccgaaatgttgtgcttgatca

SEQ ID NO: 24 - DNA, 1692 bp, synthetic construct
  misc_feature 1..1692: note = Nucleotide sequence of the P. pastoris ade2 gene
  source 1..1692: mol_type = other DNA
atggattctcaggtaataggtattctaggaggaggccagctaggccgaatgattgttgaggccgctagcaggctcaatatcaagaccgtgattcttgatgatggtttttcacctgctaagcacattaatgctgcgcaagaccacatcgacggatcattcaaagatgaggaggctatcgccaagttagctgccaaatgtgatgttctcactgtagagattgagcatgtcaacacagatgctctaaagagagttcaagacagaactggaatcaagatatatcctttaccagagacaatcgaactaatcaaggataagtacttgcaaaaggaacatttgatcaagcacaacatttcggtgacaaagtctcagggtatagaatctaatgaaaaggcgctgcttttgtttggagaagagaatggatttccatatctgttgaagtcccggactatggcttatgatggaagaggcaattttgtagtggagtctaaagaggacatcagtaaggcattagaattcttgaaagatcgtccattgtatgccgagaagtttgctccttttgttaaagaattagcggtaatggttgtgagatcactggaaggcgaagtattctcctacccaaccgtagaaactgtgcacaaggacaatatctgtcatattgtgtatgctccggccagagttaatgacaccatccaaaagaaagctcaaatattagctgaaaacactgtgaagactttcccaggcgctggaatcttcggagttgagatgttcctattgtctgatggagaacttcttgtaaatgagattgctccaaggccccacaattctggtcactatacaatcgatgcatgtgtaacatctcagttcgaagcacatgtaagagccataactggtctgccaatgccactagatttcaccaaactatctacttccaacaccaacgctattatgctcaatgttttgggtgctgaaaaatctcacggggaattagagttttgtagaagagccttagaaacacccggtgcttctgtatatctgtacggaaagaccacccgattggctcgtaagatgggtcatatcaacataataggatcttccatgttggaagcagaacaaaagttagagtacattctagaagaatcaacccacttaccatccagtactgtatcagctgacactaaaccgttggttggagttatcatgggttcagactctgatctacctgtgatttcgaaaggttgcgatattttaaaacagtttggtgttccattcgaagttactattgtctctgctcatagaacaccacagagaatgaccagatatgcctttgaagccgctagtagaggtatcaaggctatcattgcaggtgctggtggtgctgctcatcttccaggaatggttgctgccatgactccgttgccagtcattggtgttcctgtcaagggctctacgttggatggtgtagactcgctacactcgattgtccaaatgcctagaggtgttcctgtggctacggttgctatcaacaacgccaccaatgccgctctgttggccatcaggattttaggtacaattgaccacaaatggcaaaaggaaatgtccaagtatatgaatgcaatggagaccgaagtgttggggaaggcatccaacttggaatctgaagggtatgaatcctatttgaagaatcgtctttga

SEQ ID NO: 25 - DNA, 7742 bp, synthetic construct
  misc_feature 1..7742: note = Nucleotide sequence of the CRISPR/BEC10-Pp all-in-one-vectorsystem
  source 1..7742: mol_type = other DNA
atgtgagcaaaaggccagcaaaaggccaggaaccgtaaaaaggccgcgttgctggcgtttttccataggctccgcccccctgacgagcatcacaaaaatcgacgctcaagtcagaggtggcgaaacccgacaggactataaagataccaggcgtttccccctggaagctccctcgtgcgctctcctgttccgaccctgccgcttaccggatacctgtccgcctttctcccttcgggaagcgtggcgctttctcatagctcacgctgtaggtatctcagttcggtgtaggtcgttcgctccaagctgggctgtgtgcacgaaccccccgttcagcccgaccgctgcgccttatccggtaactatcgtcttgagtccaacccggtaagacacgacttatcgccactggcagcagccactggtaacaggattagcagagcgaggtatgtaggcggtgctacagagttcttgaagtggtggcctaactacggctacactagaagaacagtatttggtatctgcgctctgctgaagccagttaccttcggaaaaagagttggtagctcttgatccggcaaacaaaccaccgctggtagcggtggtttttttgtttgcaagcagcagattacgcgcagaaaaaaaggatctcaagaagatcctttgatcttttctacggggtctgacgctcagtggtacctgcagctaaggtaatcagatccaagtttccccaatcttccggggcaaaccaattcaggcaatgtggtcccacgataaggccgaatataacggccacagaagcttctccgatatagagcttctctttaataaaaagagagcacagagaaaatattgtggaaaaaacacctatacatgcgtaggcaatatgggttttggagggcgctaagtgctcccatatagccatgttgtaaaggattatgcaaaatttggcaggagaatctgtggatgcaaggtataattataccgaagggaaaaaaagagagaagagcataaaaagcttatttttagttgacgttcgcggacatagattgctggcttgataagataggacttttggatagttacagaatataagggcataaatagataataaaacatccgtatacatacaataaaactaataaatactctctaaataatcgtaaggtgtcaattgttagaaaaactcatcgagcatcaaatgaaactgcaatttattcatatcaggattatcaataccatatttttgaaaaagccgtttctgtaatgaaggagaaaactcaccgaggcagttccataggatggcaagatcctggtatcggtctgcgattccgactcgtccaacatcaatacaacctattaatttcccctcgtcaaaaataaggttatcaagtgagaaatcaccatgagtgacgactgaatccggtgagaatggcaaaagcttatgcatttctttccagacttgttcaacaggccagccattacgctcgtcatcaaaatcactcgcatcaaccaaaccgttattcattcgtgattgcgcctgagcgagacgaaatacgcgatcgctgttaaaaggacaattacaaacaggaatcgaatgcaaccggcgcaggaacactgccagcgcatcaacaatattttcacctgaatcaggatattcttctaatacctggaatgctgttttgccggggatcgcagtggtgagtaaccatgcatcatcaggagtacggataaaatgcttgatggtcggaagaggcataaattccgtcagccagtttagtctgaccatctcatctgtaacatcattggcaacgctacctttgccatgtttcagaaacaactctggcgcatcgggcttcccatacaatcgatagattgtcgcacctgattgcccgacattatcgcgagcccatttatacccatataaatcagcatccatgttggaatttaatcgcggcctcgaaacgtgagtcttttccttacccatggtttagtcctccttacaccttgtcgtattatacgagccggaagtataaagtaacaacactctagaaaattttttcggataattttttaaagcgagaaagtcacccagcggatatgaacgcttattgtgtgccgcacatcatattggcgtttgaagtcgcggtttcgagattatctcttaatttgttcgcattttactttcaagcgcaacacaatgaagtgctctaatattacaaagattgttggaactggctcacttggaattgcaacaggcgtccttgggtatgcatgcttacgcggaatcgacaaccttgtcacgttgatcgataacaacaaactggaccaacgaatgcgaaggttagtaggacgcgttcttagatccacacggtacattgttgccatatgcatgactactggatcttatctgctagtagaaactttcagaagatcacctgccagtgctcgacacttatacctgatttatgccagtcttggtgctcctacgcttgcactttactacgggtggaatgtttggcctctggaaacaactattctaaagaaactttcacgaagtcaaaatggctcaccactgcaacaaaagaaacaagacattactgaaggatcccgccggtggataagctgggggaacattcgcgaaaatgaaacaagtcggctgttatagtatatttattataatattgaaagatctcaaaagactacttatttttgaatgaaccaagtatgaaatcaacctatttggggttgaccaaaataagtaaatattaattgcgccggtgggatccgcacaaacgaaggtctcacttaatcttctgtactctgaagaggagtgggaaataccaagaaaaacatcaaactcgaatgattttcccaaacccctaccacaagatattcatctgctgcgagataggctgatcaggagcaagctcgtacgagaagaaacaaaatgacaaaaaaaatcctatactatataggttacaaataaaaaagtatcaaaaatgaagcctgcatctctcaggcaaatggcattctgacatcctcttgagcggccgcttacttcatctgaatcaagttttcgacggacttcaaggcaatatggtaagcaccattatcatcaccattgtggatgtagtggatgttgttttccctttctttcaactgtgagtcggacctaaaaccacattctttacagaccaggatgtcatccttatctctgtaaacgttagtcttagagcaaactggacacttcttagatgtgaactttggatcgatgaaatgaacaacaccgaatggcttagacttgtacttagtctcttccaacttgatgatatttctgtagttatcggcggatctaaaagctggaacaaatctcaaaacggtgttatcagattggatcttctgcagctttttcagcagctgcatttcaaaaaattggtaagtacccaagccagccaacatttgattctgctgttctttaaagtcaacatcctcatcttgagaggtggatggcaaatatctaccatcataaccagattttgcaccaccgtaagctctggacaaatcttctaaagaaatgtaggccttgtaggagtacttggcgaaaatgtagttaacgataccgatcatgttagcaacgataccttgtttcaaattgtcggcagcatccaattcgatgatcttgtttttctcagtctgattgtttcctctggcaataacaccttgcaagtcagagatcatttccctcatggtgttaataggcaaatcagcgtacttttgaccttcaccgaatgaagaaatcaagccctcgatcctctttttgaattcttcatcagatggttcgttgttgatcaggtccaagacatcttgttcattggtctgcatcttgtgttgcaactttctaatgtaggacagctgcttcaacttaatcttctgcttgttttcttcggtagcttcttcatctggagtatctctgttcttcttgaccagtgtcaaagattgatcaaccaacaccttattatcctcaatggtagtttcaactctcaagttagacaagtccaagatatgtctggtttcagccaaggtgtgcttccagtaattcttagatctcttttcggctctgacgaactcttttttgtagatttcaaagtcacccaaaatcttacccctcttgtccaaaacacacaaagtagctaattgcttcaagcctctgtcgataccaataacaacgtattctttacccaacaaggcatggttaacctttttgttgaactcttcgacggcttctttttgagcatcttcgtcgttgaagttctcgatctgcttcttcaagttgatgaactcaccattttgtgggatgatttcgcagttaaaagcgcaaacgaattgcaatctaccgtatcttttatcctttgggtagtccttaattggagttctgtaagaaacggcgaattctggatgcaatctgaattctttggaaccttcgaagatttgcttccaatccttggagaactgattcttgtccttacgaccttgagaggtgatgtcctggttgataattggcaacaacaaacaaccaccttcaaccaaagaagcaatagattgcttggaaatggtatgcttttgcaagatgtaagacttctgatcgatttcgtgttcgatatcttcgtaggagttacacttctcgaagttccaaccaaattcagcccaattttgattcttagccatggtagaatcggtcaagcaatccttaacgtattgcaacaagacttgttctctcttgtagttgtcccattctttcttgatcttggtccaatcaacatggatcttagaagtatggaaatcagcatatggagaaattgcacccttcttggtggtatgattcttaatcagcttgatcagggtcttagaggtcaaagacttaacttggtaggtgatgaattcggatgaggtgttcaacttacccaaaatggcttcgacatggttgatttgttcgtgttgcaaaccgttggccaacaagtatctgtctttgttgttatcttcgatgataataccgaaatgggtgatcttggtgatgttgttcttttctttgaacttgtctctcaattcagcgaaggttttaccgtaggtagaagagatttgcttgaattcgttggtcaacttagtgtatgggttttcgtagtaggacttgatcttaccgtacttgtcttttctgaacatcttttgagccttgattctacctttcagaccacctctaataaaacccaactgttgtttagcatcggtgtacttttcgtgacctctaccatcgttaatccaggccaagatatccttcttgtaggtttcgaactctttaatcttgtatggcagaacgatgttctcgaaggtgttgttaatcttgcagatgaattcctcttgattagatggcaggttgttcttgtgctccaaaacagccaaattctttctgatgtacaacaggtcggcgtagaacttaaaaactggttctttggagacttcgcaatcaaaaacatccttcaagtacttctcgcactgttcttttgggaaagtaacagtagtgtagacaccgttagccaattgttcccatgcgtaatcaaaagcaaccttgattgggtagtgattcaagtcaaaaacatcttcattatgagcgtaatcatgagctggagatctagtagcaccaattgcatccaaaaccttcaaaacggcatcttcatcttcagcgatatacttagccaattcgtgcttgaccaaaaatggaatgggcttgtacttaaagcattgggttctaatgataacggagatgtttctatcatcgtagatcttgaacttgtcgaacttggaaaagtactcttcgatttgcttggacgtcttgttcttcaacttttcgaccaactcaatcaacttcaactcacggatcttggcatcaatatcgttcttgaaaacgtgtggcttttgttcagcagtgtaatggttcaaggtaaccttagcaaatggagtataaccaccattggtagcaatagcatccttcaattcaccaatagaaccaaccaaatcggagtaatcgttcagagcgaattcaatcaaatgtctggattcttcaccatcttccaacttggagatgtttggaaaagaaatagcaccgttggacaatgggatgacaatttcgttaaccaagttggccaaaatggagaaggtcttgttgaagttaatcaggtttggcttggtatgagccttatcagaattttccaaagctctcttgtactgcttcaattgttgagagaaatccttcaggaaagacttttgtctggcaatgttgtccttccagtagttggtaatatgttgagatctcttcaaaccctggtaaacgttgtgcttagaagataaggatgacaaggtgatcagttgagagttttgatcaccaacatcgaatctggcctttctagccaattgtctataccagtccttgtagacggcaatttggttagttctacagtagatttgaccccaagcttcatggaacttgataatttcggagtagcacctttcgcactttttgaccaattcgatttcgttcaaggattcagcaatggtagcagatgacttcaaggtcttgtaggaaatgtcaacgaattcttgcaattccaagtgggacttgcactttttcttatcctctttcaaagtggcaccgaatctcaaagtcttagaaatttggcaggagttttcgaaggacttcatcaccttccttttctttttgggagccatgtttcggaattctgttgtagttttaatatagtttgagtatgagatggaactcagaacgaaggaattatcaccagtttatatattctgaggaaagggtgtgtcctaaattggacagtcacgatggcaataaacgctcagccaatcagaatgcaggagccataaattgttgtattattgctgcaagatttatgtgggttcacattccactgaatggttttcactgtagaattggtgtcctagttgttatgtttcgagatgttttcaagaaaaactaaaatgcacaaactgaccaataatgtgccgtcgcgcttggtacaaacgtcaggattgccaccacttttttcgcactctggtacaaaagttcgcacttcccactcgtatgtaacgaaaaacagagcagtctatccagaacgagacaaattagcgcgtactgtcccattccataaggtatcataggaaacgagagtcctccccccatcacgtatatataaacacactgatatcccacatccgcttgtcaccaaactaatacatccagttcaagttacctaaacaaatcagatcgaaattctgatgagtccgtgaggacgaaacgagtaagctcgtcaatttctactgttgtagattcaccgaaatgttgtgcttgatcaggccggcatggtcccagcctcctcgctggcgccggctgggcaacatgcttcggcatggcgaatgggactcaagaggatgtcagaatgccatttgcctgagagatgcaggcttcatttttgatacttttttatttgtaacctatatagtataggattttttttgaaatgaataataactgtgtatttttcagtgttcccgatctgcgtctatttcacaataccaacatgagtcaaccaaatccaaatgtcatcattgtaggcgatggagatttcaggcagtcaaagcgggaattggatctgggtaccgcaggaaagaac

SEQ ID NO: 26 - DNA, 4107 bp, synthetic construct
  misc_feature 1..4107: note = Nucleotide sequence of the Codon Optimized SpCas9 Sequence foryeast
  source 1..4107: mol_type = other DNA
atggacaagaagtactccatcggtttggatattggtacaaattctgttggttgggccgttattactgatgagtacaaagttccatccaagaagttcaaggttttgggtaacactgataggcactccatcaaaaagaatttgattggtgccttgttgttcgactctggtgaaactgctgaagctactagattgaaaagaaccgctagaagaagatacaccagaagaaagaacagaatctgctacttgcaagagatcttctctaacgaaatggccaaggttgatgattcattcttccacagattggaagagtccttcttggttgaagaggataagaaacacgaaagacatccaatcttcggtaacatcgttgatgaagttgcttaccacgaaaagtacccaactatctaccatttgagaaagaagttggttgactctaccgataaggctgatttgagattgatctatttggctttggcccacatgattaagttcagaggtcatttcttgatcgagggtgatttgaatccagataactccgatgttgacaagttgttcatccaattggtccaaacttacaaccagttgttcgaagaaaatccaatcaatgcctctggtgttgatgctaaggctattttgtctgctagactgtctaagtctagaaggttggaaaacttgattgctcaattgccaggtgaaaagaagaatggtttgttcggtaatttgatcgccttgtctttgggtttgactccaaatttcaagtccaacttcgatttggctgaagatgctaagttgcaattgtctaaggatacctacgatgatgacttggataatttgttggcccaaatcggtgatcaatacgctgatttgtttttggctgctaagaacttgtccgatgccattttgttgtccgatatcttgagagttaacaccgaaattactaaggctccattgtctgcctctatgatcaaaagatacgatgaacaccaccaagacttgactttgttgaaagctttggtcagacaacagttgccagaaaagtacaaagaaatcttcttcgaccagtccaaaaatggttacgctggttatattgatggtggtgcttctcaagaagagttctacaagttcattaagcccatcttggaaaagatggatggtactgaagaactgttggtcaagttgaacagagaagatttgttgagaaagcagagaaccttcgataacggttctattccacatcaaatccacttgggtgaattgcatgctattttgagaaggcaagaggatttctacccattcttgaaggataacagagaaaagatcgagaagatcctgaccttcagaattccatattatgttggtccattggccagaggtaattctagatttgcttggatgactaggaagtccgaagaaactattactccatggaacttcgaagaggttgttgataagggtgcttctgctcaatccttcattgaaagaatgactaacttcgacaagaacctgccaaacgaaaaggttttgccaaaacactctttgctgtacgaatacttcaccgtctacaacgaattgactaaggttaagtacgtcaccgaaggtatgagaaaaccagcttttttgtctggtgaacaaaagaaggctatcgtcgatttgttgttcaagactaacagaaaggttaccgtcaagcaattgaaagaggactacttcaagaaaatcgagtgcttcgattccgttgaaatttccggtgttgaagatagattcaacgcttccttaggtacttaccatgacctgttgaaaatcatcaaggacaaggatttcttggacaacgaagaaaacgaggatatcttggaggatatcgttttgactttgaccttgttcgaggatagggaaatgatcgaagaaaggttgaaaacctacgctcacttgtttgatgataaggtcatgaagcagttgaagagaagaaggtatactggttggggtagattgtctaggaaattgattaacggtatcagggacaagcaatccggtaagactattttggactttttgaagtctgatggcttcgccaatagaaacttcatgcaattgatccacgatgacagcttgaccttcaaagaagatattcaaaaggcccaagtttccggtcaaggtgattctttacatgaacatattgctaacttggctggttccccagctattaagaaaggtattttacaaaccgttaaggtggtcgacgaattggtaaaagttatgggtagacataagccagagaacatcgttattgaaatggctagagaaaatcagactacccaaaagggtcaaaagaactccagagaaaggatgaagagaattgaagagggtatcaaagaattgggctcccagattttgaaagaacacccagttgaaaacacccaattgcagaacgaaaagctgtacttgtactacttgcagaatggtagagatatgtacgtcgaccaagaattggatatcaacagattgtccgattacgatgtcgatcatatcgttccacagtcttttttgaaggatgactccatcgataacaaggtcttgactagatccgataagaacagaggtaagtctgataacgttccatctgaagaggtcgtcaagaagatgaagaattattggagacagttgctgaacgccaagttgattactcaaagaaagttcgacaatttgaccaaggctgaaagaggtggtttgtctgaattggacaaagcaggtttcattaagaggcaattggttgaaactaggcaaatcaccaaacacgttgcccaaattttggattccagaatgaataccaagtacgacgaaaacgataagttgatcagggaagttaaggtcatcacgttgaagtctaagttggtttccgatttcagaaaggacttccaattctacaaggtcagggaaatcaacaactaccatcatgctcatgatgcttacttgaatgctgttgttggtactgccttgattaagaagtatccaaagttggaatccgagttcgtttacggtgattacaaggtttacgacgtcagaaagatgattgccaagtccgaacaagaaattggtaaggctactgccaagtactttttctactccaacatcatgaatttcttcaagaccgaaatcactttggccaacggtgaaattagaaaaaggccattgattgagactaacggtgagactggtgaaatagtttgggataagggtagagatttcgctaccgttagaaaagttttgtccatgccacaagttaacatcgtcaaaaagaccgaagttcaaactggtggtttctccaaagaatccatcttgccaaaaagaaactccgacaaattgatcgccagaaagaaagattgggacccaaaaaagtatggcggttttgattctccaactgttgcttactctgttttggttgttgccaaagtcgaaaagggtaagagtaagaagttgaagtcagtcaaagagttgttgggtatcacgatcatggaaaggtcatctttcgaaaagaatcctatcgactttttggaagccaagggttacaaagaagtcaaaaaggacctgattatcaagctgccaaagtactctttgttcgaattggaaaacggtcgtaagagaatgttggcttctgctggtgaactacaaaaaggtaatgaattggctctgccctctaagtacgttaacttcttgtacttggcttctcactacgaaaagttgaaaggttctccagaagataacgagcaaaagcagttgtttgtggaacaacataagcactacttggacgaaatcatcgaacagatctctgaattctccaagagggttattttggctgatgccaatttggataaggtcttgtctgcttacaacaagcacagagataagccaattagagaacaagccgaaaacatcattcacctgttcactttgactaatttgggtgctccagctgcttttaagtacttcgatacaaccatcgacagaaagagatacacctctaccaaagaagttttggacgctaccttgatccatcaatctattactggtctgtacgaaaccagaatcgacttgtctcaattaggtggtgattaa

SEQ ID NO: 27 - DNA, 20 bp, synthetic construct
  misc_feature 1..20: note = Ade2 target-specific 24 bps spacer sequence (Cas9)
  source 1..20: mol_type = other DNA
aagagagttcaagacagaac

SEQ ID NO: 28 - DNA, 80 bp, synthetic construct
  misc_feature 1..80: note = Nucleotide sequence of the SpCas9 specific sgRNA sequence
  source 1..80: mol_type = other DNA
gttttagagctagaaatagcaagttaaaataaggctagtccgttatcaacttgaaaaagtggcaccgagtcggtgctttt

SEQ ID NO: 29 - DNA, 8210 bp, synthetic construct
  misc_feature 1..8210: note = Nucleotide sequence of the CRISPR/Cas9-Pp all-in-one-vectorsystem
  source 1..8210: mol_type = other DNA
atgtgagcaaaaggccagcaaaaggccaggaaccgtaaaaaggccgcgttgctggcgtttttccataggctccgcccccctgacgagcatcacaaaaatcgacgctcaagtcagaggtggcgaaacccgacaggactataaagataccaggcgtttccccctggaagctccctcgtgcgctctcctgttccgaccctgccgcttaccggatacctgtccgcctttctcccttcgggaagcgtggcgctttctcatagctcacgctgtaggtatctcagttcggtgtaggtcgttcgctccaagctgggctgtgtgcacgaaccccccgttcagcccgaccgctgcgccttatccggtaactatcgtcttgagtccaacccggtaagacacgacttatcgccactggcagcagccactggtaacaggattagcagagcgaggtatgtaggcggtgctacagagttcttgaagtggtggcctaactacggctacactagaagaacagtatttggtatctgcgctctgctgaagccagttaccttcggaaaaagagttggtagctcttgatccggcaaacaaaccaccgctggtagcggtggtttttttgtttgcaagcagcagattacgcgcagaaaaaaaggatctcaagaagatcctttgatcttttctacggggtctgacgctcagtggtacctgcagctaaggtaatcagatccaagtttccccaatcttccggggcaaaccaattcaggcaatgtggtcccacgataaggccgaatataacggccacagaagcttctccgatatagagcttctctttaataaaaagagagcacagagaaaatattgtggaaaaaacacctatacatgcgtaggcaatatgggttttggagggcgctaagtgctcccatatagccatgttgtaaaggattatgcaaaatttggcaggagaatctgtggatgcaaggtataattataccgaagggaaaaaaagagagaagagcataaaaagcttatttttagttgacgttcgcggacatagattgctggcttgataagataggacttttggatagttacagaatataagggcataaatagataataaaacatccgtatacatacaataaaactaataaatactctctaaataatcgtaaggtgtcaattgttagaaaaactcatcgagcatcaaatgaaactgcaatttattcatatcaggattatcaataccatatttttgaaaaagccgtttctgtaatgaaggagaaaactcaccgaggcagttccataggatggcaagatcctggtatcggtctgcgattccgactcgtccaacatcaatacaacctattaatttcccctcgtcaaaaataaggttatcaagtgagaaatcaccatgagtgacgactgaatccggtgagaatggcaaaagcttatgcatttctttccagacttgttcaacaggccagccattacgctcgtcatcaaaatcactcgcatcaaccaaaccgttattcattcgtgattgcgcctgagcgagacgaaatacgcgatcgctgttaaaaggacaattacaaacaggaatcgaatgcaaccggcgcaggaacactgccagcgcatcaacaatattttcacctgaatcaggatattcttctaatacctggaatgctgttttgccggggatcgcagtggtgagtaaccatgcatcatcaggagtacggataaaatgcttgatggtcggaagaggcataaattccgtcagccagtttagtctgaccatctcatctgtaacatcattggcaacgctacctttgccatgtttcagaaacaactctggcgcatcgggcttcccatacaatcgatagattgtcgcacctgattgcccgacattatcgcgagcccatttatacccatataaatcagcatccatgttggaatttaatcgcggcctcgaaacgtgagtcttttccttacccatggtttagtcctccttacaccttgtcgtattatacgagccggaagtataaagtaacaacactctagaaaattttttcggataattttttaaagcgagaaagtcacccagcggatatgaacgcttattgtgtgccgcacatcatattggcgtttgaagtcgcggtttcgagattatctcttaatttgttcgcattttactttcaagcgcaacacaatgaagtgctctaatattacaaagattgttggaactggctcacttggaattgcaacaggcgtccttgggtatgcatgcttacgcggaatcgacaaccttgtcacgttgatcgataacaacaaactggaccaacgaatgcgaaggttagtaggacgcgttcttagatccacacggtacattgttgccatatgcatgactactggatcttatctgctagtagaaactttcagaagatcacctgccagtgctcgacacttatacctgatttatgccagtcttggtgctcctacgcttgcactttactacgggtggaatgtttggcctctggaaacaactattctaaagaaactttcacgaagtcaaaatggctcaccactgcaacaaaagaaacaagacattactgaaggatcccgccggtggataagctgggggaacattcgcgaaaatgaaacaagtcggctgttatagtatatttattataatattgaaagatctcaaaagactacttatttttgaatgaaccaagtatgaaatcaacctatttggggttgaccaaaataagtaaatattaattgcgccggtgggatccgcacaaacgaaggtctcacttaatcttctgtactctgaagaggagtgggaaataccaagaaaaacatcaaactcgaatgattttcccaaacccctaccacaagatattcatctgctgcgagataggctgatcaggagcaagctcgtacgagaagaaacaaaatgacaaaaaaaatcctatactatataggttacaaataaaaaagtatcaaaaatgaagcctgcatctctcaggcaaatggcattctgacatcctcttgagcggccgcctagtcgcctccaagctggctcaggtcgatcctggtctcatacaggccggtaatggactggtggatcaaggtggcatccagcacctccttagtgctagtgtaccttttcctgtcgatggtggtatcgaagtatttgaatgccgcaggtgcgcccagatttgtcagggtgaacaggtgtatgatattctcggcctgctccctgatgggtttgtctcggtgcttgttgtaggcgctgaggaccttatccaggttcgcgtcggccagaatcaccctcttgctgaactcgctgatttgctcgattatctcgtccaggtaatgcttgtgctgctccacgaacagctgcttctgctcgttgtcctcggggctgcctttcagcttttcgtagtgggacgccaggtacagaaaattcacgtacttgctgggcagcgccagttcgttgcccttttgcagttccccagcgctcgccagcatcctctttctgccgttctccaattcaaacagggagtacttggggagtttgatgatcaggtcctttttgacctctttgtagcccttggcttccaaaaagtcaatggggttcttctcaaagctggacctctccatgatggttatgccgagcagctccttcacgctcttcagtttcttgctcttccccttctctaccttcgcgaccaccagcacgctgtaggctacggtggggctgtcgaagcctccatacttcttagggtcccagtccttcttccgggcgatcagcttgtcgctgttcctcttgggcaggatggattccttgctaaagccgcctgtctgcacctcagtttttttcacaatattcacctggggcatgctcaggactttcctcacggtggcgaagtccctgcccttgtcccacacgatctcgccggtctcaccgttggtctcgataagcggcctcttcctgatttcgccgttggcaagtgtgatctcggtcttgaaaaagttcatgatgttgctgtagaagaaatacttagcggtggccttgccgatctcctgttcgctcttagcgatcatcttcctcacatcgtaaactttgtagtcgccgtagacaaattcggactccagctttggatacttcttaatcagggcggtgccgaccacggcgttcaggtatgcgtcgtgggcatggtggtagttgttgatctccctcaccttgtagaactggaaatctttgcgaaagtcggacaccaacttgctcttcagggtaatcactttcacttccctgatgagtttgtcattctcatcgtacttggtattcattctgctgtcgaggatttgggccacgtgcttcgtgatctgtcgggtctcgaccagctgcctctttatgaagcccgctttgtcaagttcggagagtccgcccctctcggccttggtcaggttatcgaactttctctgggtgatcaatttcgcgttgagcagttgcctccagtagttcttcatctttttaaccacctcttcgcttggcacgttgtcgcttttgcccctgtttttgtcggagcgggtcaggaccttgttgtcgatgctatcgtctttaagaaagctctggggcactatgtgatccacgtcatagtctgaaagcctgttgatgtccaactcctggtcaacgtacatgtccctgccgttctgcaggtagtacaggtacagcttctcgttctggagctgggtattctccacggggtgctctttgaggatctggcttccgagttccttgataccctcctcgatccttttcatgcgctcccggctgttcttctggcccttttgggtggtctggttctctctggccatctctataactatgttttcgggcttgtgcctgcccatgaccttgaccaattcgtccacaaccttaacggtctgcagtatgcccttcttgatcgcaggggagcctgccaggtttgcaatatgttcgtgcagggagtcgccctggccgctaacctgggccttctggatgtcctccttgaaggtcaagctgtcatcgtgaatcagctgcatgaagtttcggttggcgaagccgtcggacttcaggaaatccaggatggtcttgccgctctgcttgtccctaatgccgttgatgagcttcctggacagtctgccccagccggtgtatcttcgtctcttcagttgtttcatcactttgtcgtcgaacaggtgggcgtaggttttgagcctttcttcaatcatctctcggtcctcaaacagggtcaaagtcagcacgatgtcctcgagtatatcctcgttctcctcattatccaggaaatccttgtctttgattatcttcaacaagtcgtggtaggtgcccaggctggcgttgaacctgtcctccacgccgcttatttccacgctatcaaagcactcgatcttcttgaagtagtcctccttcagctgcttcacggtcaccttcctgttggtcttgaacagcaggtccacgatggccttcttctgctcgccgctcaggaaagcgggttttcgcatgccctcggtcacatatttcaccttggtgagctcgttgtacacggtgaagtactcgtaaagcaggctgtgcttgggcagcaccttctcgttaggcaggtttttgtcgaaattggtcatccgttcgatgaaagactgcgcgcttgctcctttgtccaccacttcctcgaagttccagggggtgatggtctcctcgctctttcttgtcatccaagcgaatcggctgttgcccctggcaagagggcccacgtagtaggggatcctgaaggtcagaatcttttcgattttctccctattgtccttgaggaaggggtagaaatcctcctgtcgcctcagtattgcgtgcagctcgcccaggtggatctggtgggggatgctaccgttgtcaaaggtcctctgcttccggagcaaatcttccctgttcagcttcaccagcagctcctcggtgccatccatcttctccaggatgggcttgatgaacttgtagaactcctcttggctggctccgccgtcgatgtagccggcgtagccgttcttgctctggtcgaaaaagatctccttgtacttctcgggcagttgctgcctcaccagggccttcagaagggtcaggtcctgatggtgctcgtcgtacctcttgatcatgctggcgctcaggggggccttggtgatctctgtgttcaccctaaggatatcgctaagcaggattgcgtcagaaaggttcttggcggcgaggaacaggtcagcgtactggtcgccgatttgggcgagcagattgtccaagtcgtcgtcataggtgtccttactcaactgcagcttggcatcttctgccaggtcgaagttgctcttgaagttgggggtcaggcccaggctcagggcaatcagattaccgaagaggccgttcttcttttcaccgggcagctgggctatcaggttctccaagcgcctgcttttgctcagcctggcgctaagtatggccttcgcatccaccccgctggcgttaatagggttttcctcgaacagctggttataggtctgtacaagctggatgaacaatttgtctacgtcactgttgtcggggttaaggtcgccctcgatcaggaagtggcccctgaacttaatcatgtgcgccagagccaagtagataagtcgcaagtcggctttatcggtgctatccaccaatttctttcgcaggtggtagatggtggggtacttctcgtgataagcgacctcgtcgactatgttgccgaagatggggtgtcgttcgtgcttcttatcctcctcgacaaggaagctctcctccagcctgtggaagaagctgtcgtccaccttggccatctcgttgctgaagatctcctgcagatagcagatcctgttcttcctccgggtgtaccttcgccttgcggtcctcttcaacctggtggcctcggcggtctcgcctgagtcaaacagcagagccccgataaggtttttcttgatagagtgcctgtctgtattccccagcaccttgaacttcttgctgggtaccttgtattcgtctgtgataacggcccagcccacgctattggtgccgatatcaaggccgatgctgtactttttgtccatcaccttccttttctttttgggagccatgtttcggaattctgttgtagttttaatatagtttgagtatgagatggaactcagaacgaaggaattatcaccagtttatatattctgaggaaagggtgtgtcctaaattggacagtcacgatggcaataaacgctcagccaatcagaatgcaggagccataaattgttgtattattgctgcaagatttatgtgggttcacattccactgaatggttttcactgtagaattggtgtcctagttgttatgtttcgagatgttttcaagaaaaactaaaatgcacaaactgaccaataatgtgccgtcgcgcttggtacaaacgtcaggattgccaccacttttttcgcactctggtacaaaagttcgcacttcccactcgtatgtaacgaaaaacagagcagtctatccagaacgagacaaattagcgcgtactgtcccattccataaggtatcataggaaacgagagtcctccccccatcacgtatatataaacacactgatatcccacatccgcttgtcaccaaactaatacatccagttcaagttacctaaacaaatcagatctctcttctgatgagtccgtgaggacgaaacgagtaagctcgtcaagagagttcaagacagaacgttttagagctagaaatagcaagttaaaataaggctagtccgttatcaacttgaaaaagtggcaccgagtcggtgcttttggccggcatggtcccagcctcctcgctggcgccggctgggcaacatgcttcggcatggcgaatgggactcaagaggatgtcagaatgccatttgcctgagagatgcaggcttcatttttgatacttttttatttgtaacctatatagtataggattttttttgaaatgaataataactgtgtatttttcagtgttcccgatctgcgtctatttcacaataccaacatgagtcaaccaaatccaaatgtcatcattgtaggcgatggagatttcaggcagtcaaagcgggaattggatctgggtaccgcaggaaagaac

SEQ ID NO: 30 - DNA, 1998 bp, synthetic construct
  misc_feature 1..1998: note = Nucleotide sequence of the Ade2 HDR-template for BEC10 and SpCas9
  source 1..1998: mol_type = other DNA
ctggaacaagggaattcacggtaataccttttggagcaagttcaaccgatagagccttcattaatgagttgattgcacctttggtggtcgcatataccgattgattcgggtaggtcacttcgaaactgtacagggaggcagtaaagatgatcctacccttaatctggttcttaataaagtgtttagtgactagctgtgtcaatctaaatggaaaatcgacatttaccttttggatagccgcgtaatctttctccgtaaaacttgtaaactcagatttaatggcaatggcagcgttgttgattaaaatgtcaatctttccagtggaactcttctccaccgcaggactcgttacggtctcttccagctttgcaagatcggcatccactagatccaactcaattgtatgtatggaggcaccatcggcatttgacattctcacctcttcaatgaaagccgttgggtctgtagaaggtctatggataagaataagttctgcacctgcttcataaagtcctcgaactattccttggcctaatccgctggtaccaccggtgatcaaggcgaccttaccattcaaagaaaacaaatcagcggacattagcgacttgaatagggaatgggttagacaaatgaaagccgacgagccagcactttatagtaagtgcaggtgagtcaataagaataaatgtatggcttgctgtccctatcgcgtaagaagcttactaagatcgcctaaattgaaaagttgaacaaatcagttctagctggcctccatcagcatttcgttctcctctgatcatctttgccaatcgctagcatgccctcagcgtgcaaggaaaagcacgcttctttcttatcgacgtattttcaactatggcagagccaggttagcaagtcaaagccgtatactcggtagtgtgctcgccaaaaataaatttgacttgactcttcactagcctatgcaaataaggttaccttttccaagaatcgtagaaacgattaaaaaacttccaaactctcatttagtattgttttttaatagatgtatatataatagtacacgtaacttatctattccattcataattttattttaaaggttcggtagaaatttgtcctccaaaaagttggttagagcctggcagttttgataggcattattatagattgggtaatatttaccctgcacctggaggaactttgcaaagagcctcatgtgctctaaaaggatgtcagaattccaacatttcaaaattatatctgcatgcgtctgtaatactggaactgttatttttctggtcaggatttcaccgctcttgtcgtcatgtttctcgtcgtctgaaagtaaactgactttcctctttccataaacacaaaaatcgattgcaacttggttattcttgagattgaaatttgctgtgtcttcagtgcttagctgaatatcaacaaacttacttagtactaataacgaagcactatggtaagtggcataacatagtggtattgaagcgaacagtggatattgaacccaagcattggcaacatctggctctgttgatactgatccggatcgtttggcaccaattcctgaaacggcgtagtgccaccaaggtttcgatttgagaacaggttcatcatcagagtcaaccaccccaatgtcaatggcaggctccaacgaagtaggtccaacaacaacaggaagtatttgaccttgaagatctgttcctttatgatccaccacaccttgccccaattccaataactttaccagtcccgatgcagacatgataactggtactaatgatctccattgattttcgtcggcactacgtaaagcctccaaaaatgaattcagaatatcttctgaaactagattctgcttctgtgattcaagcattgctttatgtagacatctcttgaataaaagcaattctccacatattggtgtgtgtaagatagatctggaaagatgtatctggaatagtccagtcaacgttg

SEQ ID NO: 31 - DNA, 453 bp, Pichia pastoris
  source 1..453: mol_type = genomic DNA; note = Nucleotid sequence of the 453 bps L-rhamnose-inducible P. pastoris LRA4 promoter
tttgagagattttaattcaacgaactacagagtcatcaacaacgttgaaaactacgatttgatctacgaatctgggaatgtcacagcatccagcccttttgacgaatctcacatcaagaaagtccaaatcttgcctcacaattgtacgaattttacgttttccgaactgacagcctctaggtatgtcttatttgagttcacagatgttctaggttacccccaagattattcatatggagcccaagtagccgaagttgttctctactaacgaccttacgtaacgaaatatcccccatctttagattaaatgaaaaagttttgtttgttattacataatctcagtaggttgtcgcatcatccggggtaatgtcgcaccgaaatctggggattccctctgtaacccaccagtataaataatgaacagttctaccagcttcccggttactccaacca

SEQ ID NO: 32 - DNA, 24 bp, Pichia pastoris
  source 1..24: mol_type = genomic DNA; note = Nucleotide sequence of the 24 bps AOX1 target-specific spacer sequence (Info: PAM TTC)
ggggatagccatcgtttcgaataa

SEQ ID NO: 33 - DNA, 373 bp, Pichia pastoris
  source 1..373: mol_type = genomic DNA; note = Nucleotide sequence of the 373 bps RNA Pol-III promoter/tRNA sequence PtRNA1-tRNA1 from P. pastoris
ttttgtagctttataagcagctttttcttgaagcttaagtagagtagtgtgaaaaagagaccaagtacaaaatatccaccttctgggttttagtatttgtgctgagccgcatgtgttgataagaggcgataaggtacagaaatgatttgctagcaatccatcattattgaagtgtgagtgggcacctgatatcatggcttgtttattcaatagagtctgacatagtgaaagggagttatgaaattgaagaagactccatggcaggcatatgtaaatataccagccaatcctactacattgatccgtgatagtttagtggtagaaccaccgcttgtcgcgcggtagaccggggttcaattccccgtcgcggagc

SEQ ID NO: 34 - DNA, 85 bp, Pichia pastoris
  source 1..85: mol_type = genomic DNA; note = Nucleotide sequence of the 85 bps tRNA4 sequence from P. pastoris
ggcaacgtggccgagtggttaaggcgaaagattagaaatcttttgggctctgcccgcgcaggttcgagtcctgccgttgtcgtca

SEQ ID NO: 35 - DNA, 1992 bp, Pichia pastoris
  source 1..1992: mol_type = genomic DNA; note = Nucleotide sequence of the 1992 bps P. pastoris AOX1 coding gene, start and stop codons are included in the coding sequence
atggctatccccgaagagtttgatatcctagttctaggtggtggatccagtggatcctgtattgccggaagattggcaaacttggaccactccttgaaagttggtcttatcgaagcaggtgagaacaacctcaacaacccatgggtctaccttccaggtatttacccaagaaacatgaagttggactccaagactgcttccttctacacttctaacccatctcctcacttgaatggtagaagagccattgttccatgtgctaacgtcttgggtggtggttcttctatcaacttcatgatgtacaccagaggttctgcttctgattacgatgacttccaagccgagggctggaaaaccaaggacttgcttccattgatgaaaaagactgagacctaccaaagagcttgcaacaaccctgacattcacggtttcgaaggtccaatcaaggtttctttcggtaactacacctacccagtttgccaggacttcttgagggcttctgagtcccaaggtattccatacgttgacgacttggaagacttggttactgctcacggtgctgaacactggttgaagtggatcaacagagacactggtcgtcgttccgactctgctcatgcatttgtccactctactatgagaaaccacgacaacttgtacttgatctgtaacacgaaggtcgacaaaattattgtcgaagacggaagagctgctgctgttagaaccgttccaagcaagcctttgaacccaaagaagccaagtcacaagatctaccgtgctagaaagcaaatcgttttgtcttgtggtaccatctcctctccattggttttgcaaagatccggttttggtgacccaatcaagttgagagccgctggtgttaagcctttggtcaacttgccaggtgtcggaagaaacttccaagaccactactgtttcttcagtccttacagaatcaagcctcagtacgagtctttcgatgacttcgtccgtggtgatgctgagattcaaaagagagtctttgaccaatggtacgccaatggtactggtcctcttgccactaacggtatcgaagctggtgtcaagatcagaccaacaccagaagaactctctcaaatggacgaatccttccaggagggttacagagaatacttcgaagacaagccagacaagccagttatgcactactccatcattgctggtttcttcggtgaccacaccaagattcctcctggaaagtacatgactatgttccacttcttggaatacccattctccagaggttccattcacattacctccccagacccatacgcagctccagacttcgacccaggtttcatgaacgatgaaagagacatggctcctatggtttgggcttacaagaagtctagagaaaccgctagaagaatggaccactttgccggtgaggtcacttctcaccaccctctgttcccatactcatccgaggccagagccttggaaatggatttggagacctctaatgcctacggtggacctttgaacttgtctgctggtcttgctcacggttcttggactcaacctttgaagaagccaactgcaaagaacgaaggccacgttacttcgaaccaggtcgagcttcatccagacatcgagtacgatgaggaggatgacaaggccattgagaactacattcgtgagcacactgagaccacatggcactgtctgggaacctgttccatcggtccaagagaaggttccaagatcgtcaaatggggtggtgttttggaccacagatccaacgtttacggagtcaagggcttgaaggttggtgacttgtccgtgtgcccagacaatgttggttgtaacacctacaccaccgctcttttgatcggtgaaaagactgccactttggttggagaagatttaggatactctggtgaggccttagacatgactgttcctcagttcaagttgggcacttacgagaagaccggtcttgctagattctaa

SEQ ID NO: 36 - DNA, 501 bp, synthetic construct
  source 1..501: mol_type = other DNA; note = Nucleotide sequence of the 501 bps tRNA RNA Pol III promoter-mediated gRNA (gRNA) expression cassette
ttttgtagctttataagcagctttttcttgaagcttaagtagagtagtgtgaaaaagagaccaagtacaaaatatccaccttctgggttttagtatttgtgctgagccgcatgtgttgataagaggcgataaggtacagaaatgatttgctagcaatccatcattattgaagtgtgagtgggcacctgatatcatggcttgtttattcaatagagtctgacatagtgaaagggagttatgaaattgaagaagactccatggcaggcatatgtaaatataccagccaatcctactacattgatccgtgatagtttagtggtagaaccaccgcttgtcgcgcggtagaccggggttcaattccccgtcgcggagcaatttctactgttgtagatggggatagccatcgtttcgaataaggcaacgtggccgagtggttaaggcgaaagattagaaatcttttgggctctgcccgcgcaggttcgagtcctgccgttgtcgtca

SEQ ID NO: 37 - DNA, 7621 bp, synthetic construct
  source 1..7621: mol_type = other DNA; note = Nucleotide sequence of the 7621 bps CRISPR/BEC10-Pp-i vector system
atgtgagcaaaaggccagcaaaaggccaggaaccgtaaaaaggccgcgttgctggcgtttttccataggctccgcccccctgacgagcatcacaaaaatcgacgctcaagtcagaggtggcgaaacccgacaggactataaagataccaggcgtttccccctggaagctccctcgtgcgctctcctgttccgaccctgccgcttaccggatacctgtccgcctttctcccttcgggaagcgtggcgctttctcatagctcacgctgtaggtatctcagttcggtgtaggtcgttcgctccaagctgggctgtgtgcacgaaccccccgttcagcccgaccgctgcgccttatccggtaactatcgtcttgagtccaacccggtaagacacgacttatcgccactggcagcagccactggtaacaggattagcagagcgaggtatgtaggcggtgctacagagttcttgaagtggtggcctaactacggctacactagaagaacagtatttggtatctgcgctctgctgaagccagttaccttcggaaaaagagttggtagctcttgatccggcaaacaaaccaccgctggtagcggtggtttttttgtttgcaagcagcagattacgcgcagaaaaaaaggatctcaagaagatcctttgatcttttctacggggtctgacgctcagtggtacctgcagctaaggtaatcagatccaagtttccccaatcttccggggcaaaccaattcaggcaatgtggtcccacgataaggccgaatataacggccacagaagcttctccgatatagagcttctctttaataaaaagagagcacagagaaaatattgtggaaaaaacacctatacatgcgtaggcaatatgggttttggagggcgctaagtgctcccatatagccatgttgtaaaggattatgcaaaatttggcaggagaatctgtggatgcaaggtataattataccgaagggaaaaaaattttgtagctttataagcagctttttcttgaagcttaagtagagtagtgtgaaaaagagaccaagtacaaaatatccaccttctgggttttagtatttgtgctgagccgcatgtgttgataagaggcgataaggtacagaaatgatttgctagcaatccatcattattgaagtgtgagtgggcacctgatatcatggcttgtttattcaatagagtctgacatagtgaaagggagttatgaaattgaagaagactccatggcaggcatatgtaaatataccagccaatcctactacattgatccgtgatagtttagtggtagaaccaccgcttgtcgcgcggtagaccggggttcaattccccgtcgcggagcaatttctactgttgtagatggggatagccatcgtttcgaataaggcaacgtggccgagtggttaaggcgaaagattagaaatcttttgggctctgcccgcgcaggttcgagtcctgccgttgtcgtcatttttttttttttgtatacatacaataaaactaataaatactctctaaataatcgtaaggtgtcaattgttagaaaaactcatcgagcatcaaatgaaactgcaatttattcatatcaggattatcaataccatatttttgaaaaagccgtttctgtaatgaaggagaaaactcaccgaggcagttccataggatggcaagatcctggtatcggtctgcgattccgactcgtccaacatcaatacaacctattaatttcccctcgtcaaaaataaggttatcaagtgagaaatcaccatgagtgacgactgaatccggtgagaatggcaaaagcttatgcatttctttccagacttgttcaacaggccagccattacgctcgtcatcaaaatcactcgcatcaaccaaaccgttattcattcgtgattgcgcctgagcgagacgaaatacgcgatcgctgttaaaaggacaattacaaacaggaatcgaatgcaaccggcgcaggaacactgccagcgcatcaacaatattttcacctgaatcaggatattcttctaatacctggaatgctgttttgccggggatcgcagtggtgagtaaccatgcatcatcaggagtacggataaaatgcttgatggtcggaagaggcataaattccgtcagccagtttagtctgaccatctcatctgtaacatcattggcaacgctacctttgccatgtttcagaaacaactctggcgcatcgggcttcccatacaatcgatagattgtcgcacctgattgcccgacattatcgcgagcccatttatacccatataaatcagcatccatgttggaatttaatcgcggcctcgaaacgtgagtcttttccttacccatggtttagtcctccttacaccttgtcgtattatacgagccggaagtataaagtaacaacactctagaaaattttttcggataattttttaaagcgagaaagtcacccagcggatatgaacgcttattgtgtgccgcacatcatattggcgtttgaagtcgcggtttcgagattatctcttaatttgttcgcattttactttcaagcgcaacacaatgaagtgctctaatattacaaagattgttggaactggctcacttggaattgcaacaggcgtccttgggtatgcatgcttacgcggaatcgacaaccttgtcacgttgatcgataacaacaaactggaccaacgaatgcgaaggttagtaggacgcgttcttagatccacacggtacattgttgccatatgcatgactactggatcttatctgctagtagaaactttcagaagatcacctgccagtgctcgacacttatacctgatttatgccagtcttggtgctcctacgcttgcactttactacgggtggaatgtttggcctctggaaacaactattctaaagaaactttcacgaagtcaaaatggctcaccactgcaacaaaagaaacaagacattactgaaggatcccgccggtggataagctgggggaacattcgcgaaaatgaaacaagtcggctgttatagtatatttattataatattgaaagatctcaaaagactacttatttttgaatgaaccaagtatgaaatcaacctatttggggttgaccaaaataagtaaatattaattgcgccggtgggatccgcacaaacgaaggtctcacttaatcttctgtactctgaagaggagtgggaaataccaagaaaaacatcaaactcgaatgattttcccaaacccctaccacaagatattcatctgctgcgagataggctgatcaggagcaagctcgtacgagaagaaacaaaatgacaaaaaaaatcctatactatataggttacaaataaaaaagtatcaaaaatgaagcctgcatctctcaggcaaatggcattctgacatcctcttgagcggccgcttacttcatctgaatcaagttttcgacggacttcaaggcaatatggtaagcaccattatcatcaccattgtggatgtagtggatgttgttttccctttctttcaactgtgagtcggacctaaaaccacattctttacagaccaggatgtcatccttatctctgtaaacgttagtcttagagcaaactggacacttcttagatgtgaactttggatcgatgaaatgaacaacaccgaatggcttagacttgtacttagtctcttccaacttgatgatatttctgtagttatcggcggatctaaaagctggaacaaatctcaaaacggtgttatcagattggatcttctgcagctttttcagcagctgcatttcaaaaaattggtaagtacccaagccagccaacatttgattctgctgttctttaaagtcaacatcctcatcttgagaggtggatggcaaatatctaccatcataaccagattttgcaccaccgtaagctctggacaaatcttctaaagaaatgtaggccttgtaggagtacttggcgaaaatgtagttaacgataccgatcatgttagcaacgataccttgtttcaaattgtcggcagcatccaattcgatgatcttgtttttctcagtctgattgtttcctctggcaataacaccttgcaagtcagagatcatttccctcatggtgttaataggcaaatcagcgtacttttgaccttcaccgaatgaagaaatcaagccctcgatcctctttttgaattcttcatcagatggttcgttgttgatcaggtccaagacatcttgttcattggtctgcatcttgtgttgcaactttctaatgtaggacagctgcttcaacttaatcttctgcttgttttcttcggtagcttcttcatctggagtatctctgttcttcttgaccagtgtcaaagattgatcaaccaacaccttattatcctcaatggtagtttcaactctcaagttagacaagtccaagatatgtctggtttcagccaaggtgtgcttccagtaattcttagatctcttttcggctctgacgaactcttttttgtagatttcaaagtcacccaaaatcttacccctcttgtccaaaacacacaaagtagctaattgcttcaagcctctgtcgataccaataacaacgtattctttacccaacaaggcatggttaacctttttgttgaactcttcgacggcttctttttgagcatcttcgtcgttgaagttctcgatctgcttcttcaagttgatgaactcaccattttgtgggatgatttcgcagttaaaagcgcaaacgaattgcaatctaccgtatcttttatcctttgggtagtccttaattggagttctgtaagaaacggcgaattctggatgcaatctgaattctttggaaccttcgaagatttgcttccaatccttggagaactgattcttgtccttacgaccttgagaggtgatgtcctggttgataattggcaacaacaaacaaccaccttcaaccaaagaagcaatagattgcttggaaatggtatgcttttgcaagatgtaagacttctgatcgatttcgtgttcgatatcttcgtaggagttacacttctcgaagttccaaccaaattcagcccaattttgattcttagccatggtagaatcggtcaagcaatccttaacgtattgcaacaagacttgttctctcttgtagttgtcccattctttcttgatcttggtccaatcaacatggatcttagaagtatggaaatcagcatatggagaaattgcacccttcttggtggtatgattcttaatcagcttgatcagggtcttagaggtcaaagacttaacttggtaggtgatgaattcggatgaggtgttcaacttacccaaaatggcttcgacatggttgatttgttcgtgttgcaaaccgttggccaacaagtatctgtctttgttgttatcttcgatgataataccgaaatgggtgatcttggtgatgttgttcttttctttgaacttgtctctcaattcagcgaaggttttaccgtaggtagaagagatttgcttgaattcgttggtcaacttagtgtatgggttttcgtagtaggacttgatcttaccgtacttgtcttttctgaacatcttttgagccttgattctacctttcagaccacctctaataaaacccaactgttgtttagcatcggtgtacttttcgtgacctctaccatcgttaatccaggccaagatatccttcttgtaggtttcgaactctttaatcttgtatggcagaacgatgttctcgaaggtgttgttaatcttgcagatgaattcctcttgattagatggcaggttgttcttgtgctccaaaacagccaaattctttctgatgtacaacaggtcggcgtagaacttaaaaactggttctttggagacttcgcaatcaaaaacatccttcaagtacttctcgcactgttcttttgggaaagtaacagtagtgtagacaccgttagccaattgttcccatgcgtaatcaaaagcaaccttgattgggtagtgattcaagtcaaaaacatcttcattatgagcgtaatcatgagctggagatctagtagcaccaattgcatccaaaaccttcaaaacggcatcttcatcttcagcgatatacttagccaattcgtgcttgaccaaaaatggaatgggcttgtacttaaagcattgggttctaatgataacggagatgtttctatcatcgtagatcttgaacttgtcgaacttggaaaagtactcttcgatttgcttggacgtcttgttcttcaacttttcgaccaactcaatcaacttcaactcacggatcttggcatcaatatcgttcttgaaaacgtgtggcttttgttcagcagtgtaatggttcaaggtaaccttagcaaatggagtataaccaccattggtagcaatagcatccttcaattcaccaatagaaccaaccaaatcggagtaatcgttcagagcgaattcaatcaaatgtctggattcttcaccatcttccaacttggagatgtttggaaaagaaatagcaccgttggacaatgggatgacaatttcgttaaccaagttggccaaaatggagaaggtcttgttgaagttaatcaggtttggcttggtatgagccttatcagaattttccaaagctctcttgtactgcttcaattgttgagagaaatccttcaggaaagacttttgtctggcaatgttgtccttccagtagttggtaatatgttgagatctcttcaaaccctggtaaacgttgtgcttagaagataaggatgacaaggtgatcagttgagagttttgatcaccaacatcgaatctggcctttctagccaattgtctataccagtccttgtagacggcaatttggttagttctacagtagatttgaccccaagcttcatggaacttgataatttcggagtagcacctttcgcactttttgaccaattcgatttcgttcaaggattcagcaatggtagcagatgacttcaaggtcttgtaggaaatgtcaacgaattcttgcaattccaagtgggacttgcactttttcttatcctctttcaaagtggcaccgaatctcaaagtcttagaaatttggcaggagttttcgaaggacttcatcaccttccttttctttttgggagccattggttggagtaaccgggaagctggtagaactgttcattatttatactggtgggttacagagggaatccccagatttcggtgcgacattaccccggatgatgcgacaacctactgagattatgtaataacaaacaaaactttttcatttaatctaaagatgggggatatttcgttacgtaaggtcgttagtagagaacaacttcggctacttgggctccatatgaataatcttgggggtaacctagaacatctgtgaactcaaataagacatacctagaggctgtcagttcggaaaacgtaaaattcgtacaattgtgaggcaagatttggactttcttgatgtgagattcgtcaaaagggctggatgctgtgacattcccagattcgtagatcaaatcgtagttttcaacgttgttgatgactctgtagttcgttgaattaaaatctctcaaaac

SEQ ID NO: 38 - DNA, 2694 bp, synthetic construct
  source 1..2694: mol_type = other DNA; note = Nucleotide sequence of the 2694 bps GFP-expressing DNA Donor Template
taacatccaaagacgaaaggttgaatgaaacctttttgccatccgacatccacaggtccattctcacacataagtgccaaacgcaacaggaggggatacactagcagcagaccgttgcaaacgcaggacctccactcctcttctcctcaacacccacttttgccatcgaaaaaccagcccagttattgggcttgattggagctcgctcattccaattccttctattaggctactaacaccatgactttattagcctgtctatcctggcccccctggcgaggttcatgtttgtttatttccgaatgcaacaagctccgcattacacccgaacatcactccagatgagggctttctgagtgtggggtcaaatagtttcatgttccccaaatggcccaaaactgacagtttaaacgctgtcttggaacctaatatgacaaaagcgtgatctcatccaagatgaactaagtttggttcgttgaaatgctaacggccagttggtcaaaaagaaacttccaaaagtcggcataccgtttgtcttgtttggtattgattgacgaatgctcaaaaataatctcattaatgcttagcgcagtctctctatcgcttctgaaccccggtgcacctgtgccgaaacgcaaatggggaaacacccgctttttggatgattatgcattgtctccacattgtatgcttccaagattctggtgggaatactgctgatagcctaacgttcatgatcaaaatttaactgttctaacccctacttgacagcaatatataaacagaaggaagctgccctgtcttaaacctttttttttatcatcattattagcttactttcataattgcgactggttccaattgacaagcttttgattttaacgacttttaacgacaacttgagaagatcaaaaaacaactaattattgaaagaattccgaaacgatggctagcaaaggagaagaactcttcactggagttgtcccaattcttgttgaattagatggtgatgttaacggccacaagttctctgtcagtggagagggtgaaggtgatgcaacatacggaaaacttaccctgaagttcatctgcactactggcaaactgcctgttccatggccaacactagtcactactctgtgctatggtgttcaatgcttttcaagatacccggatcatatgaaacggcatgactttttcaagagtgccatgcccgaaggttatgtacaggaaaggaccatcttcttcaaagatgacggcaactacaagacacgtgctgaagtcaagtttgaaggtgatacccttgttaatagaatcgagttaaaaggtattgacttcaaggaagatggcaacattctgggacacaaattggaatacaactataactcacacaatgtatacatcatggcagacaaacaaaagaatggaatcaaagtgaacttcaagacccgccacaacattgaagatggaagcgttcaactagcagaccattatcaacaaaatactccaattggcgatggccctgtccttttaccagacaaccattacctgtccacacaatctgccctttcgaaagatcccaacgaaaagagagaccacatggtccttcttgagtttgtaacagctgctgggattacacatggcatggatgaactgtacaactgagcggccgctggtggatccagtggatcctgtattgccggaagattggcaaacttggaccactccttgaaagttggtcttatcgaagcaggtgagaacaacctcaacaacccatgggtctaccttccaggtatttacccaagaaacatgaagttggactccaagactgcttccttctacacttctaacccatctcctcacttgaatggtagaagagccattgttccatgtgctaacgtcttgggtggtggttcttctatcaacttcatgatgtacaccagaggttctgcttctgattacgatgacttccaagccgagggctggaaaaccaaggacttgcttccattgatgaaaaagactgagacctaccaaagagcttgcaacaaccctgacattcacggtttcgaaggtccaatcaaggtttctttcggtaactacacctacccagtttgccaggacttcttgagggcttctgagtcccaaggtattccatacgttgacgacttggaagacttggttactgctcacggtgctgaacactggttgaagtggatcaacagagacactggtcgtcgttccgactctgctcatgcatttgtccactctactatgagaaaccacgacaacttgtacttgatctgtaacacgaaggtcgacaaaattattgtcgaagacggaagagctgctgctgttagaaccgttccaagcaagcctttgaacccaaagaagccaagtcacaagatctaccgtgctagaaagcaaatcgttttgtcttgtggtaccatctcctctccattggttttgcaaagatccggttttggtgacccaatcaagttgagagccgctggtgttaagcctttggtcaacttgccaggtgtcggaagaaacttccaagaccactactgtttcttcagtccttacagaatcaagcctcagtacgagtctttcgatgacttcgtccgtggtgatgctgagattcaaaagagagtctttgaccaatggtacgccaatggtactggtcctcttgccact

SEQ ID NO: 39 - DNA, 24 bp, synthetic construct
  source 1..24: mol_type = other DNA; note = Nucleotide sequence of the 24 bps oligonucleotide PCR_AOX1_fw
tgacaccagcttcgataccgttag

SEQ ID NO: 40 - DNA, 24 bp, synthetic construct
  source 1..24: mol_type = other DNA; note = Nucleotide sequence of the 24 bps oligonucleotide PCR_AOX1_rv
catgagtcgcaaccaacctacctc